European Patent Specification EP 4 034 668 B1, published April 17, 2024. Title: METHOD FOR PRODUCING 2-METHYL-BUTYRIC ACID BY BACTERIAL FERMENTATION. Applicant: Ajinomoto Co., Inc. The sequence listing filed with the application follows.

SEQUENCE LISTING (69 sequences)

SEQ ID NO: 1 - DNA, 1194 bp, Escherichia coli
gtgtttcaaaaagttgacgcctacgctggcgacccgattcttacgcttatggagcgttttaaagaagaccctcgcagcgacaaagtgaatttaagtatcggtctgtactacaacgaagacggaattattccacaactgcaagccgtggcggaggcggaagcgcgcctgaatgcgcagcctcatggcgcttcgctttatttaccgatggaagggcttaactgctatcgccatgccattgcgccgctgctgtttggtgcggaccatccggtactgaaacaacagcgcgtagcaaccattcaaacccttggcggctccggggcattgaaagtgggcgcggatttcctgaaacgctacttcccggaatcaggcgtctgggtcagcgatcctacctgggaaaaccacgtagcaatattcgccggggctggattcgaagtgagtacttacccctggtatgacgaagcgactaacggcgtgcgctttaatgacctgttggcgacgctgaaaacattacctgcccgcagtattgtgttgctgcatccatgttgccacaacccaacgggtgccgatctcactaatgatcagtgggatgcggtgattgaaattctcaaagcccgcgagcttattccattcctcgatattgcctatcaaggatttggtgccggtatggaagaggatgcctacgctattcgcgccattgccagcgctggattacccgctctggtgagcaattcgttctcgaaaattttctccctttacggcgagcgcgtcggcggactttctgttatgtgtgaagatgccgaagccgctggccgcgtactggggcaattgaaagcaacagttcgccgcaactactccagcccgccgaattttggtgcgcaggtggtggctgcagtgctgaatgacgaggcattgaaagccagctggctggcggaagtagaagagatgcgtactcgcattctggcaatgcgtcaggaattggtgaaggtattaagcacagagatgccagaacgcaatttcgattatctgcttaatcagcgcggcatgttcagttataccggtttaagtgccgctcaggttgaccgactacgtgaagaatttggtgtctatctcatcgccagcggtcgcatgtgtgtcgccgggttaaatacggcaaatgtacaacgtgtggcaaaggcgtttgctgcggtgatgtaa

SEQ ID NO: 2 - protein, 397 aa, Escherichia coli
MFQKVDAYAGDPILTLMERFKEDPRSDKVNLSIGLYYNEDGIIPQLQAVAEAEARLNAQPHGASLYLPMEGLNCYRHAIAPLLFGADHPVLKQQRVATIQTLGGSGALKVGADFLKRYFPESGVWVSDPTWENHVAIFAGAGFEVSTYPWYDEATNGVRFNDLLATLKTLPARSIVLLHPCCHNPTGADLTNDQWDAVIEILKARELIPFLDIAYQGFGAGMEEDAYAIRAIASAGLPALVSNSFSKIFSLYGERVGGLSVMCEDAEAAGRVLGQLKATVRRNYSSPPNFGAQVVAAVLNDEALKASWLAEVEEMRTRILAMRQELVKVLSTEMPERNFDYLLNQRGMFSYTGLSAAQVDRLREEFGVYLIASGRMCVAGLNTANVQRVAKAFAAVM

SEQ ID NO: 3 - DNA, 1572 bp, Escherichia coli
atgagccagcaagtcattattttcgataccacattgcgcgacggtgaacaggcgttacaggcaagcttgagtgtgaaagaaaaactgcaaattgcgctggcccttgagcgtatgggtgttgacgtgatggaagtcggtttccccgtctcttcgccgggcgattttgaatcggtgcaaaccatcgcccgccaggttaaaaacagccgcgtatgtgcgttagctcgctgcgtggaaaaagatatcgacgtggcggccgaatccctgaaagtcgccgaagccttccgtattcatacctttattgccacttcgccaatgcacatcgccaccaagctgcgcagcacgctggacgaggtgatcgaacgcgctatctatatggtgaaacgcgcccgtaattacaccgatgatgttgaattttcttgcgaagatgccgggcgtacacccattgccgatctggcgcgagtggtcgaagcggcgattaatgccggtgccaccaccatcaacattccggacaccgtgggctacaccatgccgtttgagttcgccggaatcatcagcggcctgtatgaacgcgtgcctaacatcgacaaagccattatctccgtacatacccacgacgatttgggcctggcggtcggaaactcactggcggcggtacatgccggtgcacgccaggtggaaggcgcaatgaacgggatcggcgagcgtgccggaaactgttccctggaagaagtcatcatggcgatcaaagttcgtaaggatattctcaacgtccacaccgccattaatcaccaggagatatggcgcaccagccagttagttagccagatttgtaatatgccgatcccggcaaacaaagccattgttggcagcggcgcattcgcacactcctccggtatacaccaggatggcgtgctgaaaaaccgcgaaaactacgaaatcatgacaccagaatctattggtctgaaccaaatccagctgaatctgacctctcgttcggggcgtgcggcggtgaaacatcgcatggatgagatggggtataaagaaagtgaatataatttagacaatttgtacgatgctttcctgaagctggcggacaaaaaaggtcaggtgtttgattacgatctggaggcgctggccttcatcggtaagcagcaagaagagccggagcatttccgtctggattacttcagcgtgcagtctggctctaacgatatcgccaccgccgccgtcaaactggcctgtggcgaagaagtcaaagcagaagccgccaacggtaacggtccggtcgatgccgtctatcaggcaattaaccgcatcactgaatataacgtcgaactggtgaaatacagcctgaccgccaaaggccacggtaaagatgcgctgggtcaggtggatatcgtcgctaactacaacggtcgccgcttccacggcgtcggcctggctaccgatattgtcgagtcatctgccaaagccatggtgcacgttctgaacaatatctggcgtgccgcagaagtcgaaaaagagttgcaacgcaaagctcaacacaacgaaaacaacaaggaaaccgtgtga

SEQ ID NO: 4 - protein, 523 aa, Escherichia coli
MSQQVIIFDTTLRDGEQALQASLSVKEKLQIALALERMGVDVMEVGFPVSSPGDFESVQTIARQVKNSRVCALARCVEKDIDVAAESLKVAEAFRIHTFIATSPMHIATKLRSTLDEVIERAIYMVKRARNYTDDVEFSCEDAGRTPIADLARVVEAAINAGATTINIPDTVGYTMPFEFAGIISGLYERVPNIDKAIISVHTHDDLGLAVGNSLAAVHAGARQVEGAMNGIGERAGNCSLEEVIMAIKVRKDILNVHTAINHQEIWRTSQLVSQICNMPIPANKAIVGSGAFAHSSGIHQDGVLKNRENYEIMTPESIGLNQIQLNLTSRSGRAAVKHRMDEMGYKESEYNLDNLYDAFLKLADKKGQVFDYDLEALAFIGKQQEEPEHFRLDYFSVQSGSNDIATAAVKLACGEEVKAEAANGNGPVDAVYQAINRITEYNVELVKYSLTAKGHGKDALGQVDIVANYNGRRFHGVGLATDIVESSAKAMVHVLNNIWRAAEVEKELQRKAQHNENNKETV

SEQ ID NO: 5 - DNA, 1092 bp, Escherichia coli
atgtcgaagaattaccatattgccgtattgccgggggacggtattggtccggaagtgatgacccaggcgctgaaagtgctggatgccgtgcgcaaccgctttgcgatgcgcatcaccaccagccattacgatgtaggcggcgcagccattgataaccacgggcaaccactgccgcctgcgacggttgaaggttgtgagcaagccgatgccgtgctgtttggctcggtaggcggcccgaagtgggaacatttaccaccagaccagcaaccagaacgcggcgcgctgctgcctctgcgtaagcacttcaaattattcagcaacctgcgcccggcaaaactgtatcaggggctggaagcattctgtccgctgcgtgcagacattgccgcaaacggcttcgacatcctgtgtgtgcgcgaactgaccggcggcatctatttcggtcagccaaaaggccgcgaaggtagcggacaatatgaaaaagcctttgataccgaggtgtatcaccgttttgagatcgaacgtatcgcccgcatcgcgtttgaatctgctcgcaagcgtcgccacaaagtgacgtcgatcgataaagccaacgtgctgcaatcctctattttatggcgggagatcgttaacgagatcgccacggaatacccggatgtcgaactggcgcatatgtacatcgacaacgccaccatgcagctgattaaagatccatcacagtttgacgttctgctgtgctccaacctgtttggcgacattctgtctgacgagtgcgcaatgatcactggctcgatggggatgttgccttccgccagcctgaacgagcaaggttttggactgtatgaaccggcgggcggctcggcaccagatatcgcaggcaaaaacatcgccaacccgattgcacaaatcctttcgctggcactgctgctgcgttacagcctggatgccgatgatgcggcttgcgccattgaacgcgccattaaccgcgcattagaagaaggcattcgcaccggggatttagcccgtggcgctgccgccgttagtaccgatgaaatgggcgatatcattgcccgctatgtagcagaaggggtgtaa

SEQ ID NO: 6 - protein, 363 aa, Escherichia coli
MSKNYHIAVLPGDGIGPEVMTQALKVLDAVRNRFAMRITTSHYDVGGAAIDNHGQPLPPATVEGCEQADAVLFGSVGGPKWEHLPPDQQPERGALLPLRKHFKLFSNLRPAKLYQGLEAFCPLRADIAANGFDILCVRELTGGIYFGQPKGREGSGQYEKAFDTEVYHRFEIERIARIAFESARKRRHKVTSIDKANVLQSSILWREIVNEIATEYPDVELAHMYIDNATMQLIKDPSQFDVLLCSNLFGDILSDECAMITGSMGMLPSASLNEQGFGLYEPAGGSAPDIAGKNIANPIAQILSLALLLRYSLDADDAACAIERAINRALEEGIRTGDLARGAAAVSTDEMGDIIARYVAEGV

SEQ ID NO: 7 - DNA, 1401 bp, Escherichia coli
atggctaagacgttatacgaaaaattgttcgacgctcacgttgtgtacgaagccgaaaacgaaaccccactgttatatatcgaccgccacctggtgcatgaagtgacctcaccgcaggcgttcgatggtctgcgcgcccacggtcgcccggtacgtcagccgggcaaaaccttcgctaccatggatcacaacgtctctacccagaccaaagacattaatgcctgcggtgaaatggcgcgtatccagatgcaggaactgatcaaaaactgcaaagaatttggcgtcgaactgtatgacctgaatcacccgtatcaggggatcgtccacgtaatggggccggaacagggcgtcaccttgccggggatgaccattgtctgcggcgactcgcataccgccacccacggcgcgtttggcgcactggcctttggtatcggcacttccgaagttgaacacgtactggcaacgcaaaccctgaaacagggccgcgcaaaaaccatgaaaattgaagtccagggcaaagccgcgccgggcattaccgcaaaagatatcgtgctggcaattatcggtaaaaccggtagcgcaggcggcaccgggcatgtggtggagttttgcggcgaagcaatccgtgatttaagcatggaaggtcgtatgaccctgtgcaatatggcaatcgaaatgggcgcaaaagccggtctggttgcaccggacgaaaccacctttaactatgtcaaaggccgtctgcatgcgccgaaaggcaaagatttcgacgacgccgttgcctactggaaaaccctgcaaaccgacgaaggcgcaactttcgataccgttgtcactctgcaagcagaagaaatttcaccgcaggtcacctggggcaccaatcccggccaggtgatttccgtgaacgacaatattcccgatccggcttcgtttgccgatccggttgaacgcgcgtcggcagaaaaagcgctggcctatatggggctgaaaccgggtattccgctgaccgaagtggctatcgacaaagtgtttatcggttcctgtaccaactcgcgcattgaagatttacgcgcggcagcggagatcgccaaagggcgaaaagtcgcgccaggcgtgcaggcactggtggttcccggctctggcccggtaaaagcccaggcggaagcggaaggtctggataaaatctttattgaagccggttttgaatggcgcttgcctggctgctcaatgtgtctggcgatgaacaacgaccgtctgaatccgggcgaacgttgtgcctccaccagcaaccgtaactttgaaggccgccaggggcgcggcgggcgcacgcatctggtcagcccggcaatggctgccgctgctgctgtgaccggacatttcgccgacattcgcaacattaaataa

SEQ ID NO: 8 - protein, 466 aa, Escherichia coli
MAKTLYEKLFDAHVVYEAENETPLLYIDRHLVHEVTSPQAFDGLRAHGRPVRQPGKTFATMDHNVSTQTKDINACGEMARIQMQELIKNCKEFGVELYDLNHPYQGIVHVMGPEQGVTLPGMTIVCGDSHTATHGAFGALAFGIGTSEVEHVLATQTLKQGRAKTMKIEVQGKAAPGITAKDIVLAIIGKTGSAGGTGHVVEFCGEAIRDLSMEGRMTLCNMAIEMGAKAGLVAPDETTFNYVKGRLHAPKGKDFDDAVAYWKTLQTDEGATFDTVVTLQAEEISPQVTWGTNPGQVISVNDNIPDPASFADPVERASAEKALAYMGLKPGIPLTEVAIDKVFIGSCTNSRIEDLRAAAEIAKGRKVAPGVQALVVPGSGPVKAQAEAEGLDKIFIEAGFEWRLPGCSMCLAMNNDRLNPGERCASTSNRNFEGRQGRGGRTHLVSPAMAAAAAVTGHFADIRNIK

SEQ ID NO: 9 - DNA, 606 bp, Escherichia coli
atggcagagaaatttatcaaacacacaggcctggtggttccgctggatgccgccaatgtcgataccgatgcaatcatcccgaaacagtttttgcagaaagtgacccgtacgggttttggcgcgcatctgtttaacgactggcgttttctggatgaaaaaggccaacagccaaacccggacttcgtgctgaacttcccgcagtatcagggcgcttccattttgctggcacgagaaaacttcggctgtggctcttcgcgtgagcacgcgccctgggcattgaccgactacggttttaaagtggtgattgcgccgagttttgctgacatcttctacggcaatagctttaacaaccagctgctgccggtgaaattaagcgatgcagaagtggacgaactgtttgcgctggtgaaagctaatccggggatccatttcgacgtggatctggaagcgcaagaggtgaaagcgggagagaaaacctatcgctttaccatcgatgccttccgccgccactgcatgatgaacggtctggacagtattgggcttaccttgcagcacgacgacgccattgccgcttatgaagcaaaacaacctgcgtttatgaattaa

SEQ ID NO: 10 - protein, 201 aa, Escherichia coli
MAEKFIKHTGLVVPLDAANVDTDAIIPKQFLQKVTRTGFGAHLFNDWRFLDEKGQQPNPDFVLNFPQYQGASILLARENFGCGSSREHAPWALTDYGFKVVIAPSFADIFYGNSFNNQLLPVKLSDAEVDELFALVKANPGIHFDVDLEAQEVKAGEKTYRFTIDAFRRHCMMNGLDSIGLTLQHDDAIAAYEAKQPAFMN

SEQ ID NO: 11 - DNA, 399 bp, Artificial Sequence
  tdh::attB
tttcttctatccggtcgttccgaaaggtcaggcgcgtattcgtacccagatgtctgcggcgcatacccctgagcaaattacgcgtgcagtagaagcatttacgcgtattggtaaacaactgggcgttatcgcctgaggatgtgagatgaaagcgttatccaaactgaaagcggaagaggcgctcaagttagtataaaaaagcaggcttcaggccagtccgggaaagttattctgagctgggattaacacgaacaagggctggtattccagcccttttatctgaggataatctgttaaatatgtaaaatcctgtcagtgtaataaagagttcgtaattgtgctgatctcttatatagctgctctcattatctctctaccctgaagtgactctctcacctg

SEQ ID NO: 12 - DNA, 5991 bp, Artificial Sequence
  mini-Mu::Plac-lacI-ilvA*-kan
tgtattgattcacttgaagtacgaaaaaaaccgggaggacattggattattcgggatctgatgggattagatttggtggggcttgcaagcctgtagtgcaaattttagtcgttaatcaatgaaacgcgaaagatagtaaaaaattgcttttgtttcattgaaaatacgaaaaacaaaaacactgcaaatcatttcaataacagcttcaaaaaacgttcaaaaccgataacaaccaagctgtcaccaaatgactcatatcacaaatcagcttatgccgtttaggtatgttacatgtgtgattatgtgaggtgaagtatgttttagctggttcatggttgttatacggctttttttacctcctgtggttcctgtgaaggtactacaacactttcctgttcatgaatcccatactttgacaaaatctctttgcgtttttcttcaggtaatgcagtggtcgaaaaaaaaagcccgcactgtcaggtgcgggcttttttctgtgttaagcttgcatgcaaggagatggcgcccaacagtcccccggccacggggcctgccaccatacccacgccgaaacaagcgctcatgagcccgaagtggcgagcccgatcttccccatcggtgatgtcggcgatataggcgccagcaaccgcacctgtggcgccggtgatgccggccacgatgcgtccggcgtagaggatcgagatcctttgcctggcggcagtagcgcggtggtcccacctgaccccatgccgaactcagaagtgaaacgccgtagcgccgatggtagtgtggggtctccccatgcgagagtagggaactgccaggcatcaaataaaacgaaaggctcagtcgaaagactgggcctttcgttttatctgttgtttgtcggtgaacgctctcctgagtaggacaaatccgccgggagcggatttgaacgttgcgaagcaacggcccggagggtggcgggcaggacgcccgccataaactgccaggcatcaaattaagcagaaggccatcctgacggatggcctttttgcgtttctacaaactctttttgctgcagagatctgcgggcagtgagcgcaacgcaattaatgtgagttagctcactcattaggcaccccaggctttacactttatgcttccggctcgtataatgtgtggaattgtgagcggataacaatttcacacaggatctagaaataattttgtttaactttaagaaggagatatacatatgaaaccagtaacgttatacgatgtcgcagagtatgccggtgtctcttatcagaccgtttcccgcgtggtgaaccaggccagccacgtttctgcgaaaacgcgggaaaaagtggaagcggcgatggcggagctgaattacattcccaaccgcgtggcacaacaactggcgggcaaacagtcgttgctgattggcgttgccacctccagtctggccctgcacgcgccgtcgcaaattgtcgcggcgattaaatctcgcgccgatcaactgggtgccagcgtggtggtgtcgatggtagaacgaagcggcgtcgaagcctgtaaagcggcggtgcacaatcttctcgcgcaacgcgtcagtgggctgatcattaactatccgctggatgaccaggatgccattgctgtggaagctgcctgcactaatgttccggcgttatttcttgatgtctctgaccagacacccatcaacagtattattttctcccatgaagacggtacgcgactgggcgtggagcatctggtcgcattgggtcaccagcaaatcgcgctgttagcgggcccattaagttctgtctcggcgcgtctgcgtctggctggctggcataaatatctcactcgcaatcaaattcagccgatagcggaacgggaaggcgactggagtgccatgtccggttttcaacaaaccatgcaaatgctgaatgagggcatcgttcccactgcgatgctggttgccaacgatcagatggcgctgggcgcaatgcgcgccattaccgagtccgggctgcgcgttggtgcggatatctcggtagtgggatacgacgataccgaagacagctcatgttatatcccgccgttaaccaccatcaaacaggattttcgcctgctggggcaaaccagcgtggaccgcttgctgcaactctctcagggccaggcggtgaagggcaatcagctgttgcccgtctcactggtgaaaagaaaaaccaccctggcgcccaatacgcaaaccgcctctccccgcgcgttggccgattcattaatgcagctggcacgacaggtttcccgactggaaagcgggcagtgagcggatctcgatcccgcgaaattaatacgactcactataggggaattgtgagcggataacaattcccctctagaaataattttgtttaactttaagaaggagatatacatatggctgactcgcaacccctgtccggtgctccggaaggtgccgaatatttaagagcagtgctgcgcgcgccggtttacgaggcggcgcaggttacgccgctacaaaaaatggaaaaactgtcgtcgcgtcttgataacgtcattctggtgaagcgcgaagatcgccagccagtgcacagctttaagctgcgcggcgcatacgccatgatggcgggcctgacggaagaacagaaagcgcacggcgtgatcactgcttctgcgggtaaccacgcgcagggcgtcgcgttttcttctgcgcggttaggcgtgaaggccctgatcgttatgccaaccgccaccgccgacatcaaagtcgacgcggtgcgcggcttcggcggcgaagtgctgctcaacggcgcgaactttgatgaagcgaaagccaaagcgatcgaactgtcacagcagcaggggttcacctgggtgccgccgttcgaccatccgatggtgattgccgggcaaggcacgctggcgctggaactgctccagcaggacgcccatctcgaccgcgtatttgtgccagtcggcggcggcggtctggctgctggcgtggcggtgctgatcaaacaactgatgccgcaaatcaaagtgatcgccgtagaagcggaagactccgcctgcctgaaagcagcgctggatgcgggtcatccggttgatctgccgcgcgtagggctatttgctgaaggcgtagcggtaaaacgcatcggtgacgaaaccttccgtttatgccaggagtatctcgacgacatcatcaccgtcgatagcgatgcgatctgtgcggcgatgaaggatttattcgaagatgtgcgcgcggtggcggaaccctctggcgcgctggcgctggcgggaatgaaaaaatatatcgccctgcacaacattcgcggcgaacggctggcgcatattctttccggtgccaacgtgaacttccacggcctgcgctacgtctcagaacgctgcgaactgggcgaacagcgtgaagcgttgttggcggtgaccattccggaagaaaaaggcagcttcctcaaattctgccaactgcttggcgggcgttcggtcaccgagttcaactaccgttttgccgatgccaaaaacgcctgcatctttgtcggtgtgcgcctgagccgcggcctcgaagagcgcaaagaaattttgcagatgctcaacgacggcggctacagcgtggttgatctctccgacgacgaaatggcgaagctacacgtgcgctatatggtcggcggacgtccatcgcatccgttgcaggaacgcctctacagcttcgaattcccggaatcaccgggcgcgctgctgcgcttcctcaacacgctgggtacgtactggaacatttctttgttccactatcgcagccatggcaccgactacgggcgcgtactggcggcgttcgaacttggcgaccatgaaccggatttcgaaacccggctgaatgagctgggctacgattgccacgacgaaaccaataacccggcgttcaggttctttttggcgggttagggtccgtcgacctgcaggggggggggggaaagccacgttgtgtctcaaaatctctgatgttacattgcacaagataaaaatatatcatcatgaacaataaaactgtctgcttacataaacagtaatacaaggggtgttatgagccatattcaacgggaaacgtcttgctcgaggccgcgattaaattccaacatggatgctgatttatatgggtataaatgggctcgcgataatgtcgggcaatcaggtgcgacaatctatcgattgtatgggaagcccgatgcgccagagttgtttctgaaacatggcaaaggtagcgttgccaatgatgttacagatgagatggtcagactaaactggctgacggaatttatgcctcttccgaccatcaagcattttatccgtactcctgatgatgcatggttactcaccactgcgatccccgggaaaacagcattccaggtattagaagaatatcctgattcaggtgaaaatattgttgatgcgctggcagtgttcctgcgccggttgcattcgattcctgtttgtaattgtccttttaacagcgatcgcgtatttcgtctcgctcaggcgcaatcacgaatgaataacggtttggttgatgcgagtgattttgatgacgagcgtaatggctggcctgttgaacaagtctggaaagaaatgcataagcttttgccattctcaccggattcagtcgtcactcatggtgatttctcacttgataaccttatttttgacgaggggaaattaataggttgtattgatgttggacgagtcggaatcgcagaccgataccaggatcttgccatcctatggaactgcctcggtgagttttctccttcattacagaaacggctttttcaaaaatatggtattgataatcctgatatgaataaattgcagtttcatttgatgctcgatgagtttttctaatcagaattggttaattggttgtaacactggcagagcattacgctgacttgacgggacggcggctttgttgaataaatcgaacttttgctgagttgaaggatcagatcacgcatcttcccgacaacgcagaccgttccgtggcaaagcaaaagttcaaaatcaccaactggtccacctacaacaaagctctcatcaaccgtggctccctcactttctggctggatgatggggcgattcaggcctggtatgagtcagcaacaccttcttcacgaggcagaccttagggcccccccccccctgcaggtcgacggatccgaattctagtagaggtcgaaattcacctcgaaagcaagctgataaaccgatacaattaaaggctccttttggagcctttttttttggagattttcaacgtgaaaaaattattattcgcaattccaagctaattcacctcgaaagcaagctgataaaccgatacaattaaaggctccttttggagcctttttttttggagattttcaacgtgaaaaaattattattcgcaattccaagctctgcctcgcgcgtttcggtgatgacggtgaaaacctctgacacatgcagctcccggagacggtcacagcttgtctgtaagcggatgccgggagcagacaagcccgtcagggcgcgtcagcgggtgttggcgggtgtcggggcgcagccatgacccagtcacgtagcgatagcggagtgtatgggctcgatcccctcgcgagttggttcagctgctgcctgaggctggacgacctcgcggagttctaccggcagtgcaaatccgtcggcatccaggaaaccagcagcggctatccgcgcatccatgcccccgaacgatccccatgtaatgaataaaaagcagtaattaatacatctgtttcatttgaagcgcgaaagctaaagtttcgcatggatccccatgtaatgaataaaaagcagtaattaatacatctgtttcatttgaagcgcgaaagctaaagttttcgcatttatcgtgaaacgctttcgcgtttttcgtgcgccgcttca

SEQ ID NO: 13 - DNA, 6758 bp, Artificial Sequence
  PL-SD1-ilvG*MEDA
tgcaagtgaagttgagttgttctggcggtggaatgatgctcgcaaaaatgcagcggacaaaggatgaactacgaggaagggaacaacattcatacgctcaagttagtataaaaaagcaggcttcaagatcttcacctaccaaacaatgcccccctgcaaaaaataaattcatataaaaaacatacagataaccatctgcggtgataaattatctctggcggtgttgacataaataccactggcggtgatactgagcacatcagcaggacgcactgaccaccatgaaggtgacgctcttaaaaattaagccctgaagaagggcagcattcaaagcagaaggctttggggtgtgtgatacgaaacgaagcattggccggaaggagaactaactatgaatggcgcacagtgggtggtacatgcgttgcgggcacagggtgtgaacaccgttttcggttatccgggtggcgcaattatgccggtttacgatgcattgtatgacggcggcgtggagcacttgctatgccgacatgagcagggtgcggcaatggcggctatcggttatgctcgtgctaccggcaaaactggcgtatgtatcgccacgtctggtccgggcgcaaccaacctgataaccgggcttgcggacgcactgttagattccatccctgttgttgccatcaccggtcaagtgtccgcaccgtttatcggcactgacgcatttcaggaagtggatgtcctgggattgtcgttagcctgtaccaagcacagctttctggtgcagtcgctggaagagttgccgcgcatcatggctgaagcattcgacgttgcctgctcaggtcgtcctggtccggttctggtcgatatcccaaaagatatccagttagccagcggtgacctggaaccgtggttcaccaccgttgaaaacgaagtgactttcccacatgccgaagttgagcaagcgcgccagatgctggcaaaagcgcaaaaaccgatgctgtacgttggcggtggcgtgggtatggcgcaggcagttccggctttgcgtgaatttctcgctgccacaaaaatgcctgccacctgtacgctgaaagggctgggcgcagtagaagcagattatccgtactatctgggcatgctggggatgcacggcaccaaagcggcaaacttcgcggtgcaggagtgtgacctgctgatcgccgtgggcgcacgttttgatgaccgggtgaccggcaaactgaacaccttcgcgccacacgccagtgttatccatatggatatcgacccggcagaaatgaacaagctgcgtcaggcacatgtggcattacaaggtgatttaaatgctctgttaccagcattacagcagccgttaaatcaaaatgactggcagcaacactgcgcgcagctgcgtgatgaacattcctggcgttacgaccatcccggtgacgctatctacgcgccgttgttgttaaaacaactgtcggatcgtaaacctgcggattgcgtcgtgaccacagatgtggggcagcaccagatgtgggctgcgcagcacatcgcccacactcgcccggaaaatttcatcacctccagcggtttaggtaccatgggttttggtttaccggcggcggttggcgcacaagtcgcgcgaccgaacgataccgttgtctgtatctccggtgacggctctttcatgatgaatgtgcaagagctgggcaccgtaaaacgcaagcagttaccgttgaaaatcgtcttactcgataaccaacggttagggatggttcgacaatggcagcaactgttttttcaggaacgatacagcgaaaccacccttactgataaccccgatttcctcatgttagccagcgccttcggcatccatggccaacacatcacccggaaagaccaggttgaagcggcactcgacaccatgctgaacagtgatgggccatacctgcttcatgtctcaatcgacgaacttgagaacgtctggccgctggtgccgcctggcgccagtaattcagaaatgttggagaaattatcatgatgcaacatcaggtcaatgtatcggctcgcttcaatccagaaaccttagaacgtgttttacgcgtggtgcgtcatcgtggtttccacgtctgctcaatgaatatggccgccgccagcgatgcacaaaatataaatatcgaattgaccgttgccagcccacggtcggtcgacttactgtttagtcagttaaataaactggtggacgtcgcacacgttgccatctgccagagcacaaccacatcacaacaaatccgcgcctgagcgcaaaaggaatataaaaatgaccacgaagaaagctgattacatttggttcaatggggagatggttcgctgggaagacgcgaaggtgcatgtgatgtcgcacgcgctgcactatggcacttcggtttttgaaggcatccgttgctacgactcgcacaaaggaccggttgtattccgccatcgtgagcatatgcagcgtctgcatgactccgccaaaatctatcgcttcccggtttcgcagagcattgatgagctgatggaagcttgtcgtgacgtgatccgcaaaaacaatctcaccagcgcctatatccgtccgctgatcttcgtcggtgatgttggcatgggagtaaacccgccagcgggatactcaaccgacgtgattatcgctgctttcccgtggggagcgtatctgggcgcagaagcgctggagcaggggatcgatgcgatggtttcctcctggaaccgcgcacgaccaaacaccatcccgacggcggcaaaagccggtggtaactacctctcttccctgctggtgggtagcgaagcgcgccgccacggttatcaggaaggtatcgcgctggatgtgaacggttatatctctgaaggcgcaggcgaaaacctgtttgaagtgaaagatggtgtgctgttcaccccaccgttcacctcctccgcgctgccgggtattacccgtgatgccatcatcaaactggcgaaagagctgggaattgaagtacgtgagcaggtgctgtcgcgcgaatccctgtacctggcggatgaagtgtttatgtccggtacggcggcagaaatcacgccagtgcgcagcgtagacggtattcaggttggcgaaggccgttgtggcccggttaccaaacgcattcagcaagccttcttcggcctcttcactggcgaaaccgaagataaatggggctggttagatcaagttaatcaataaatacaaaaaatgggacggcacgcaccgtcccatttacgagacagacactgggagtaaataaagtatgcctaagtaccgttccgccaccaccactcatggtcgtaatatggcgggtgctcgtgcgctgtgggcccaccggaatgaccgacgccgatttcggtaagccgattatcgcggttgtgaactcgttcacccaatttgtaccgggtcacgtccatctgcgcgatctcggtaaactggtcgccgaacaaattgaagcggctggcggcgttgccaaagagttcaacaccattgcggtggatgatgggattgccatgggccacggggggatgctttattcactgccatctcgcgaactgatcgctgattccgttgagtatatggtcaacgcccactgcgccgacgccatggtctgcatctctaactgcgacaaaatcaccccggggatgctgatggcttccctgcgcctgaatattccggtgatctttgtttccggcggcccgatggaggccgggaaaaccaaactttccgatcagatcatcaagctcgatctggttgatgcgatgatccagggcgcagacccgaaagtatctgactcccagagcgatcaggttgaacgttccgcgtgtccgacctgcggttcctgctccgggatgtttaccgctaactcaatgaactgcctgaccgaagcgctgggcctgtcgcagccgggcaacggctcgctgctggcaacccacgccgaccgtaagcagctgttccttaatgctggtaaacgcattgttgaattgaccaaacgttattacgagcaaaacgacgaaagtgcactgccgcgtaatatcgccagtaaggcggcgtttgaaaacgccatgacgctggatatcgcgatgggtggatcgactaacaccgtacttcacctgctggcggcggcgcaggaagcggaaatcgacttcaccatgagtgatatcgataagctttcccgcaaggttccacagctgtgtaaagttgcgccgagcacccagaaataccatatggaagatgttcaccgtgctggtggtgttatcggtattctcggcgaactggatcgcgcggggttactgaaccgtgatgtgaaaaacgtacttggcctgacgttgccgcaaacgctggaacaatacgacgttatgctgacccaggatgacgcggtaaaaaatatgttccgcgcaggtcctgcaggcattcgtaccacacaggcattctcgcaagattgccgttgggatacgctggacgacgatcgcgccaatggctgtatccgctcgctggaacacgcctacagcaaagacggcggcctggcggtgctctacggtaactttgcggaaaacggctgcatcgtgaaaacggcaggcgtcgatgacagcatcctcaaattcaccggcccggcgaaagtgtacgaaagccaggacgatgcggtagaagcgattctcggcggtaaagttgtcgccggagatgtggtagtaattcgctatgaaggcccgaaaggcggtccggggatgcaggaaatgctctacccaaccagcttcctgaaatcaatgggtctcggcaaagcctgtgcgctgatcaccgacggtcgtttctctggtggcacctctggtctttccatcggccacgtctcaccggaagcggcaagcggcggcagcattggcctgattgaagatggtgacctgatcgctatcgacatcccgaaccgtggcattcagttacaggtaagcgatgccgaactggcggcgcgtcgtgaagcgcaggacgctcgaggtgacaaagcctggacgccgaaaaatcgtgaacgtcaggtctcctttgccctgcgtgcttatgccagcctggcaaccagcgccgacaaaggcgcggtgcgcgataaatcgaaactggggggttaataatggctgactcgcaacccctgtccggtgctccggaaggtgccgaatatttaagagcagtgctgcgcgcgccggtttacgaggcggcgcaggttacgccgctacaaaaaatggaaaaactgtcgtcgcgtcttgataacgtcattctggtgaagcgcgaagatcgccagccagtgcacagctttaagctgcgcggcgcatacgccatgatggcgggcctgacggaagaacagaaagcgcacggcgtgatcactgcttctgcgggtaaccacgcgcagggcgtcgcgttttcttctgcgcggttaggcgtgaaggccctgatcgttatgccaaccgccaccgccgacatcaaagtcgacgcggtgcgcggcttcggcggcgaagtgctgctccacggcgcgaactttgatgaagcgaaagccaaagcgatcgaactgtcacagcagcaggggttcacctgggtgccgccgttcgaccatccgatggtgattgccgggcaaggcacgctggcgctggaactgctccagcaggacgcccatctcgaccgcgtatttgtgccagtcggcggcggcggtctggctgctggcgtggcggtgctgatcaaacaactgatgccgcaaatcaaagtgatcgccgtagaagcggaagactccgcctgcctgaaagcagcgctggatgcgggtcatccggttgatctgccgcgcgtagggctatttgctgaaggcgtagcggtaaaacgcatcggtgacgaaaccttccgtttatgccaggagtatctcgacgacatcatcaccgtcgatagcgatgcgatctgtgcggcgatgaaggatttattcgaagatgtgcgcgcggtggcggaaccctctggcgcgctggcgctggcgggaatgaaaaaatatatcgccctgcacaacattcgcggcgaacggctggcgcatattctttccggtgccaacgtgaacttccacggcctgcgctacgtctcagaacgctgcgaactgggcgaacagcgtgaagcgttgttggcggtgaccattccggaagaaaaaggcagcttcctcaaattctgccaactgcttggcgggcgttcggtcaccgagttcaactaccgttttgccgatgccaaaaacgcctgcatctttgtcggtgtgcgcctgagccgcggcctcgaagagcgcaaagaaattttgcagatgctcaacgacggcggctacagcgtggttgatctctccgacgacgaaatggcgaagctacacgtgcgctatatggtcggcggacgtccatcgcatccgttgcaggaacgcctctacagcttcgaattcccggaatcaccgggcgcgctgctgcgcttcctcaacacgctgggtacgtactggaacatttctttgttccactatcgcagccatggcaccgactacgggcgcgtactggcggcgttcgaacttggcgaccatgaaccggatttcgaaacccggctgaatgagctgggctacgattgccacgacgaaaccaataacccggcgttcaggttctttttggcgggttagggaaaaatgcctgatagcgcttcgcttatcaggcctacccgcgcgacaacg

SEQ ID NO: 14 - DNA, 6498 bp, Artificial Sequence
  dacA::mini-Mu::cat-Pthr-attB-thrA*BC
agcttttcattctgactgcaacgggcaatatgtctctgtgtggattaaaaaaagagtgtctgatagcagcttctgaactggttacctgccgtgagtaaattaaaattttattgacttaggtcactaaatactttaaccaatataggcatagcgcacagacagataaagactctagagtccgaccaaaggtaacgaggtaacaaccatgcgagtgttgaagttcggcggtacatcagtggcaaatgcagaacgttttctgcgtgttgccgatattctggaaagcaatgccaggcaggggcaggtggccaccgtcctctctgcccccgccaaaatcaccaaccacctggtggcgatgattgaaaaaaccattagcggccaggatgctttacccaatatcagcgatgccgaacgtatttttgccgaacttttgacgggactcgccgccgcccagccggggttcccgctggcgcaattgaaaactttcgtcgatcaggaatttgcccaaataaaacatgtcctgcatggcattagtttgttggggcagtgcccggatagcatcaacgctgcgctgatttgccgtggcgagaaaatgtcgatcgccattatggccggcgtattagaagcgcgcggtcacaacgttactgttatcgatccggtcgaaaaactgctggcagtggggcattacctcgaatctaccgtcgatattgctgagtccacccgccgtattgcggcaagccgcattccggctgatcacatggtgctgatggcaggtttcaccgccggtaatgaaaaaggcgaactggtggtgcttggacgcaacggttccgactactctgctgcggtgctggctgcctgtttacgcgccgattgttgcgagatttggacggacgttgacggggtctatacctgcgacccgcgtcaggtgcccgatgcgaggttgttgaagtcgatgtcctaccaggaagcgatggagctttcctacttcggcgctaaagttcttcacccccgcaccattacccccatcgcccagttccagatcccttgcctgattaaaaataccggaaatcctcaagcaccaggtacgctcattggtgccagccgtgatgaagacgaattaccggtcaagggcatttccaatctgaataacatggcaatgttcagcgtttctggtccggggatgaaagggatggtcggcatggcggcgcgcgtctttgcagcgatgtcacgcgcccgtatttccgtggtgctgattacgcaatcatcttccgaatacagcatcagtttctgcgttccacaaagcgactgtgtgcgagctgaacgggcaatgcaggaagagttctacctggaactgaaagaaggcttactggagccgctggcagtgacggaacggctggccattatctcggtggtaggtgatggtatgcgcaccttgcgtgggatctcggcgaaattctttgccgcactggcccgcgccaatatcaacattgtcgccattgctcagagatcttctgaacgctcaatctctgtcgtggtaaataacgatgatgcgaccactggcgtgcgcgttactcatcagatgctgttcaataccgatcaggttatcgaagtgtttgtgattggcgtcggtggcgttggcggtgcgctgctggagcaactgaagcgtcagcaaagctggctgaagaataaacatatcgacttacgtgtctgcggtgttgccaactcgaaggctctgctcaccaatgtacatggccttaatctggaaaactggcaggaagaactggcgcaagccaaagagccgtttaatctcgggcgcttaattcgcctcgtgaaagaatatcatctgctgaacccggtcattgttgactgcacttccagccaggcagtggcggatcaatatgccgacttcctgcgcgaaggtttccacgttgtcacgccgaacaaaaaggccaacacctcgtcgatggattactaccatcagttgcgttatgcggcggaaaaatcgcggcgtaaattcctctatgacaccaacgttggggctggattaccggttattgagaacctgcaaaatctgctcaatgcaggtgatgaattgatgaagttctccggcattctttctggttcgctttcttatatcttcggcaagttagacgaaggcatgagtttctccgaggcgaccacgctggcgcgggaaatgggttataccgaaccggacccgcgagatgatctttctggtatggatgtggcgcgtaaactattgattctcgctcgtgaaacgggacgtgaactggagctggcggatattgaaattgaacctgtgctgcccgcagagtttaacgccgagggtgatgttgccgcttttatggcgaatctgtcacaactcgacgatctctttgccgcgcgcgtggcgaaggcccgtgatgaaggaaaagttttgcgctatgttggcaatattgatgaagatggcgtctgccgcgtgaagattgccgaagtggatggtaatgatccgctgttcaaagtgaaaaatggcgaaaacgccctggccttctatagccactattatcagccgctgccgttggtactgcgcggatatggtgcgggcaatgacgttacagctgccggtgtctttgctgatctgctacgtaccctctcatggaagttaggagtctgacatggttaaagtttatgccccggcttccagtgccaatatgagcgtcgggtttgatgtgctcggggcggcggtgacacctgttgatggtgcattgctcggagatgtagtcacggttgaggcggcagagacattcagtctcaacaacctcggacgctttgccgataagctgccgtcagaaccacgggaaaatatcgtttatcagtgctgggagcgtttttgccaggaactgggtaagcaaattccagtggcgatgaccctggaaaagaatatgccgatcggttcgggcttaggctccagtgcctgttcggtggtcgcggcgctgatggcgatgaatgaacactgcggcaagccgcttaatgacactcgtttgctggctttgatgggcgagctggaaggccgtatctccggcagcattcattacgacaacgtggcaccgtgttttctcggtggtatgcagttgatgatcgaagaaaacgacatcatcagccagcaagtgccagggtttgatgagtggctgtgggtgctggcgtatccggggattaaagtctcgacggcagaagccagggctattttaccggcgcagtatcgccgccaggattgcattgcgcacgggcgacatctggcaggcttcattcacgcctgctattcccgtcagcctgagcttgccgcgaagctgatgaaagatgttatcgctgaaccctaccgtgaacggttactgccaggcttccggcaggcgcggcaggcggtcgcggaaatcggcgcggtagcgagcggtatctccggctccggcccgaccttgttcgctctgtgtgacaagccggaaaccgcccagcgcgttgccgactggttgggtaagaactacctgcaaaatcaggaaggttttgttcatatttgccggctggatacggcgggcgcacgagtactggaaaactaaatgaaactctacaatctgaaagatcacaacgagcaggtcagctttgcgcaagccgtaacccaggggttgggcaaaaatcaggggctgttttttccgcacgacctgccggaattcagcctgactgaaattgatgagatgctgaagctggattttgtcacccgcagtgcgaagatcctctcggcgtttattggtgatgaaatcccacaggaaatcctggaagagcgcgtgcgcgcggcgtttgccttcccggctccggtcgccaatgttgaaagcgatgtcggttgtctggaattgttccacgggccaacgctggcatttaaagatttcggcggtcgctttatggcacaaatgctgacccatattgcgggtgataagccagtgaccattctgaccgcgacctccggtgataccggagcggcagtggctcatgctttctacggtttaccgaatgtgaaagtggttatcctctatccacgaggcaaaatcagtccactgcaagaaaaactgttctgtacattgggcggcaatatcgaaactgttgccatcgacggcgatttcgatgcctgtcaggcgctggtgaagcaggcgtttgatgatgaagaactgaaagtggcgctagggttaaactcggctaactcgattaacatcagccgtttgctggcgcagatttgctactactttgaagctgttgcgcagctgccgcaggagacgcgcaaccagctggttgtctcggtgccaagcggaaacttcggcgatttgacggcgggtctgctggcgaagtcactcggtctgccggtgaaacgttttattgctgcgaccaacgtgaacgataccgtgccacgtttcctgcacgacggtcagtggtcacccaaagcgactcaggcgacgttatccaacgcgatggacgtgagtcagccgaacaactggccgcgtgtggaagagttgttccgccgcaaaatctggcaactgaaagagctgggttatgcagccgtggatgatgaaaccacgcaacagacaatgcgtgagttaaaagaactgggctacacttcggagccgcacgctgccgtagcttatcgtgcgctgcgtgatcagttgaatccaggcgaatatggcttgttcctcggcaccgcgcatccggcgaaatttaaagagagcgtggaagcgattctcggtgaaacgttggatctgccaaaagagctggcagaacgtgctgatttacccttgctttcacataatctgcccgccgattttgctgcgttgcgtaaattgatgatgaatcatcagtaaaatctattcattatctcaatcaggccgggtttgcttttatgcagcccggcttttttatgaagaaattatggagaaaaatgacagggaaaaaggagaaattctcaataaatgcggtaacttagagattaggattgcggagaataacaaccgccgttctcatcgagtaatctcggatatcgaccataacgggaatgataaaaggagtaacctgtgaaaaagatgcaatctatcgtactcgcactttccctggttctggtcgctcccatggcagcacaggctgcggaaattacgttagtcccgtcagtaaaattacagataggcgatcgtgataatcgtggctattactgggatggaggtcactggcgcgaccacggctggtggaaacaacattatgaatggcgaggcaatcgctggcacctacacggaccgccgccaccgccgcgccaccataagaaagctcctcatgatcatcacggcggtcatggtcctggcaaacatcaccgctaaatgacaaatgccgggtaacaatccggcattcagcgcctgatgcgacgctggcgcgtcttatcaggcctacgttaattctgcaatatattgaatctgcatgcttttgtaggcaggataaggcgttcacgccgcatccggcattgactgcaaacttaacgctgctcgtagcgtttaaacaccagttcgccattgctggaggaatcttcatcaaagaagtaaccttcgctattaaaaccagtcagttgctctggtttggtcagccgattttcaataatgaaacgactcatcagaccgcgtgctttcttagcgtagaagctgatgatcttaaatttgccgttcttctcatcgaggaacaccggcttgataatctcggcattcaatttcttcggcttcaccgatttaaaatactcatctgacgccagattaatcaccacattatcgccttgtgctgcgagcgcctcgttcagcttgttggtgatgatatctccccagaattgatacagatctttccctcgggcattctcaagacggatccccgggtaccgagctcggtacccggggatcctctagagtcgaaattcacctcgaaagcaagctgataaaccgatacaattaaaggctccttttggagcctttttttttggagattttcaacgtgaaaaaattattattcgcaattcaagctaattcacctcgaaagcaagctgataaaccgatacaattaaaggctccttttggagcctttttttttggagattttcaacgtgaaaaaattattattcgcaattctgcctcgcgcgtttcggtgatgacggtgaaaacctctgacacatgcagctcccggagacggtcacagcttgtctgtaagcggatgccgggagcagacaagcccgtcagggcgcgtcagcgggtgttggcgggtgtcggggcgcagccatgacccagtcacgtagcgatagcggagtgtatgggctcgatcccctcggatccccatgtaatgaataaaaagcagtaattaatacatctgtttcatttgaagcgcgaaagctaaagttttcgcatttatcgtgaaacgctttcgcgtttttcgtgcgccgcttca

SEQ ID NO: 15 - DNA, 21 bp, Artificial Sequence
  Primer P1
atacaaaacggcatctccgtg

SEQ ID NO: 16 - DNA, 20 bp, Artificial Sequence
  Primer P2
ctgcctggcattgctttcca

SEQ ID NO: 17 - DNA, 1256 bp, Artificial Sequence
  DNA fragment 1
atacaaaacggcatctccgtggagaatgagtaaaagtgggggaaaagtatatcacagcgaggagaggggagttacccgaccaggagccgggtaacggagaagcgagttacagaaccatgcggacaatatcgattttgcccagttcttcatacagtgtttcaacctgctcgatatgagtggcgttgatagtgatagataccgagtggtagttgcctttgctgcttggttttaccgttggggtgtagtcacctggcgcatggcgctgtaccacttcaaccacctgatcaaccagctcaggtaacgcctgccccataactttgtaagtaaaaggagtagggaattcaagcagttcgttaagtttggttttcatgtcagctccggcgtaacgtaattaaatagcaactcccgccagaaggcgggagttttttactgatgcttagtatatggggacggaaattacactttcaagtgtttaatttttaaccaaaccagtgatggaacattaatttaatgtaatgtattgattcacttgaagtacgaaaaaaaccgggaggacattggattattcgggatctgatgggattagatttggtggggcttgcaagcctgtagtgcaaattttagtcgttaatcaatgaaacgcgaaagatagtaaaaaattgcttttgtttcattgaaaatacgaaaaacaaaaacactgcaaatcatttcaataacagcttcaaaaaacgttcaaaaccgataacaaccaagctgtcaccaaatgactcatatcacaaatcagcttatgccgtttaggtatgttacatgtgtgattatgtgaggtgaagtatgttttagctggttcatggttgttatacggctttttttacctcctgtggttcctgtgaaggtactacaacactttcctgttcatgaatcccatactttgacaaaatctctttgcgtttttcttcaggtaagcttttcattctgactgcaacgggcaatatgtctctgtgtggattaaaaaaagagtgtctgatagcagcttctgaactggttacctgccgtgagtaaattaaaattttattgacttaggtcactaaatactttaaccaatataggcatagcgcacagacagataaagactctagagtccgaccaaaggtaacgaggtaacaaccatgcgagtgttgaagttcggcggtacatcagtggcaaatgcagaacgttttctgcgtgttgccgatattctggaaagcaatgccaggcag

SEQ ID NO: 18 - DNA, 2452 bp, Artificial Sequence
  DNA fragment 2
atacaaaacggcatctccgtggagaatgagtaaaagtgggggaaaagtatatcacagcgaggagaggggagttacccgaccaggagccgggtaacggagaagcgagttacagaaccatgcggacaatatcgattttgcccagttcttcatacagtgtttcaacctgctcgatatgagtggcgttgatagtgatagataccgagtggtagttgcctttgctgcttggttttaccgttggggtgtagtcacctggcgcatggcgctgtaccacttcaaccacctgatcaaccagctcaggtaacgcctgccccataactttgtaagtaaaaggagtagggaattcaagcagttcgttaagtttggttttcatgtcagctccggcgtaacgtaattaaatagcaactcccgccagaaggcgggagttttttactgatgcttagtatatggggacggaaattacactttcaagtgtttaatttttaaccaaaccagtgatggaacattaatttaatgtaatgaagcctgcttttttatactaagttggcattataaaaaagcattgcttatcaatttgttgcaacgaacaggtcactatcagtcaaaataaaatcattatttgatttcgaattctcatgtttgacagcttatcatcgataagctttaatgcggtagtttatcacagttaaattgctaacgcagtcaggcaccgtgtatgaaatctaacaatgcgctcatcgtcatcctcggcaccgtcaccctggatgctgtaggcataggcttggttatgccggtactgccgggcctcttgcgggatatcgtccattccgacagcatcgccagtcactatggcgtgctgctagcgctatatgcgttgatgcaatttctatgcgcacccgttctcggagcactgtccgaccgctttggccgccgcccagtcctgctcgcttcgctacttggagccactatcgactacgcgatcatggcgaccacacccgtcctgtggatctccggataagtagacagcctgataagtcgcacgaaaaacaggtattgacaacatgaagtaacatgcagtaagatacaaatcgctaggtaacactagcagcgtcaaccgggcgctctagctagagccaagctagcttggccggatccgagattttcaggagctaaggaagctaaaatggagaaaaaaatcactggatataccaccgttgatatatcccaatggcatcgtaaagaacattttgaggcatttcagtcagttgctcaatgtacctataaccagaccgttcagctggatattacggcctttttaaagaccgtaaagaaaaataagcacaagttttatccggcctttattcacattcttgcccgcctgatgaatgctcatccggaattccgtatggcaatgaaagacggtgagctggtgatatgggatagtgttcacccttgttacaccgttttccatgagcaaactgaaacgttttcatcgctctggagtgaataccacgacgatttccggcagtttctacacatatattcgcaagatgtggcgtgttacggtgaaaacctggcctatttccctaaagggtttattgagaatatgtttttcgtctcagccaatccctgggtgagtttcaccagttttgatttaaacgtggccaatatggacaacttcttcgcccccgttttcaccatgggcaaatattatacgcaaggcgacaaggtgctgatgccgctggcgattcaggttcatcatgccgtctgtgatggcttccatgtcggcagaatgcttaatgaattacaacagtactgcgatgagtggcagggcggggcgtaatttttttaaggcagttattggtgcccttaaacgcctggtgctacgcctgaataagtgataataagcggatgaatggcagaaattcgtcgaagcttaacacagaaaaaagcccgcacctgacagtgcgggctttttttttcgaccactgcagtctgttacaggtcactaataccatctaagtagttgattcatagtgactgcatatgttgtgttttacagtattatgtagtctgttttttatgcaaaatctaatttaatatattgatatttatatcattttacgtttctcgttcagcttttttatactaacttgagcgagcttttcattctgactgcaacgggcaatatgtctctgtgtggattaaaaaaagagtgtctgatagcagcttctgaactggttacctgccgtgagtaaattaaaattttattgacttaggtcactaaatactttaaccaatataggcatagcgcacagacagataaagactctagagtccgaccaaaggtaacgaggtaacaaccatgcgagtgttgaagttcggcggtacatcagtggcaaatgcagaacgttttctgcgtgttgccgatattctggaaagcaatgccaggcag

SEQ ID NO: 19 - DNA, 842 bp, Artificial Sequence
  DNA fragment 3
atacaaaacggcatctccgtggagaatgagtaaaagtgggggaaaagtatatcacagcgaggagaggggagttacccgaccaggagccgggtaacggagaagcgagttacagaaccatgcggacaatatcgattttgcccagttcttcatacagtgtttcaacctgctcgatatgagtggcgttgatagtgatagataccgagtggtagttgcctttgctgcttggttttaccgttggggtgtagtcacctggcgcatggcgctgtaccacttcaaccacctgatcaaccagctcaggtaacgcctgccccataactttgtaagtaaaaggagtagggaattcaagcagttcgttaagtttggttttcatgtcagctccggcgtaacgtaattaaatagcaactcccgccagaaggcgggagttttttactgatgcttagtatatggggacggaaattacactttcaagtgtttaatttttaaccaaaccagtgatggaacattaatttaatgtaatgaagcctgcttttttatactaacttgagcgagcttttcattctgactgcaacgggcaatatgtctctgtgtggattaaaaaaagagtgtctgatagcagcttctgaactggttacctgccgtgagtaaattaaaattttattgacttaggtcactaaatactttaaccaatataggcatagcgcacagacagataaagactctagagtccgaccaaaggtaacgaggtaacaaccatgcgagtgttgaagttcggcggtacatcagtggcaaatgcagaacgttttctgcgtgttgccgatattctggaaagcaatgccaggcag

SEQ ID NO: 20 - DNA, 3539 bp, Artificial Sequence
  cynX::cat-PL-ilvA*
tgcaccagtacgttttccgcagctgtgggtcaaagacgctcaagttagtataaaaaagctgaacgagaaacgtaaaatgatataaatatcaatatattaaattagattttgcataaaaaacagactacataatactgtaaaacacaacatatgcagtcactatgaatcaactacttagatggtattagtgacctgtaacagactgcagtggtcgaaaaaaaaagcccgcactgtcaggtgcgggcttttttctgtgttaagcttcgacgaatttctgccattcatccgcttattatcacttattcaggcgtagcaccaggcgtttaagggcaccaataactgccttaaaaaaattacgccccgccctgccactcatcgcagtactgttgtaattcattaagcattctgccgacatggaagccatcacagacggcatgatgaacctgaatcgccagcggcatcagcaccttgtcgccttgcgtataatatttgcccatggtgaaaacgggggcgaagaagttgtccatattggccacgtttaaatcaaaactggtgaaactcacccagggattggctgagacgaaaaacatattctcaataaaccctttagggaaataggccaggttttcaccgtaacacgccacatcttgcgaatatatgtgtagaaactgccggaaatcgtcgtggtattcactccagagcgatgaaaacgtttcagtttgctcatggaaaacggtgtaacaagggtgaacactatcccatatcaccagctcaccgtctttcattgccatacggaattccggatgagcattcatcaggcgggcaagaatgtgaataaaggccggataaaacttgtgcttatttttctttacggtctttaaaaaggccgtaatatccagctgaacggtctggttataggtacattgagcaactgactgaaatgcctcaaaatgttctttacgatgccattgggatatatcaacggtggtatatccagtgatttttttctccattttagcttccttagctcctgaaaatctcggatccgatatctagctagagcgcccggttgacgctgctagtgttacctagcgatttgtatcttactgcatgttacttcatgttgtcaatacctgtttttcgtgcgacttatcaggctgtctacttatccggagatccacaggacgggtgtggtcgccatgatcgcgtagtcgatagtggctccaagtagcgaagcgagcaggactgggcggcggccaaagcggtcggacagtgctccgagaacgggtgcgcatagaaattgcatcaacgcatatagcgctagcagcacgccatagtgactggcgatgctgtcggaatggacgatatcccgcaagaggcccggcagtaccggcataaccaagcctatgcctacagcatccagggtgacggtgccgaggatgacgatgagcgcattgttagatttcatacacggtgcctgactgcgttagcaatttaactgtgataaactaccgcattaaagcttatcgatgataagctgtcaaacatgagaattcgaaatcaaataatgattttattttgactgatagtgacctgttcgttgcaacaaattgataagcaatgcttttttataatgccaacttagtataaaaaagcaggcttcaagatcttcacctaccaaacaatgcccccctgcaaaaaataaattcatataaaaaacatacagataaccatctgcggtgataaattatctctggcggtgttgacataaataccactggcggtgatactgagcacatcagcaggacgcactgaccaccatgaaggtgacgctcttaaaaattaagccctgaagaagggcagcattcaaagcagaaggctttggggtgtgtgatacgaaacgaagcattggccggaaggagaactaactatggctgactcgcaacccctgtccggtgctccggaaggtgccgaatatttaagagcagtgctgcgcgcgccggtttacgaggcggcgcaggttacgccgctacaaaaaatggaaaaactgtcgtcgcgtcttgataacgtcattctggtgaagcgcgaagatcgccagccagtgcacagctttaagctgcgcggcgcatacgccatgatggcgggcctgacggaagaacagaaagcgcacggcgtgatcactgcttctgcgggtaaccacgcgcagggcgtcgcgttttcttctgcgcggttaggcgtgaaggccctgatcgttatgccaaccgccaccgccgacatcaaagtcgacgcggtgcgcggcttcggcggcgaagtgctgctccacggcgcgaactttgatgaagcgaaagccaaagcgatcgaactgtcacagcagcaggggttcacctgggtgccgccgttcgaccatccgatggtgattgccgggcaaggcacgctggcgctggaactgctccagcaggacgcccatctcgaccgcgtatttgtgccagtcggcggcggcggtctggctgctggcgtggcggtgctgatcaaacaactgatgccgcaaatcaaagtgatcgccgtagaagcggaagactccgcctgcctgaaagcagcgctggatgcgggtcatccggttgatctgccgcgcgtagggctatttgctgaaggcgtagcggtaaaacgcatcggtgacgaaaccttccgtttatgccaggagtatctcgacgacatcatcaccgtcgatagcgatgcgatctgtgcggcgatgaaggatttattcgaagatgtgcgcgcggtggcggaaccctctggcgcgctggcgctggcgggaatgaaaaaatatatcgccctgcacaacattcgcggcgaacggctggcgcatattctttccggtgccaacgtgaacttccacggcctgcgctacgtctcagaacgctgcgaactgggcgaacagcgtgaagcgttgttggcggtgaccattccggaagaaaaaggcagcttcctcaaattctgccaactgcttggcgggcgttcggtcaccgagttcaactaccgttttgccgatgccaaaaacgcctgcatctttgtcggtgtgcgcctgagccgcggcctcgaagagcgcaaagaaattttgcagatgctcaacgacggcggctacagcgtggttgatctctccgacgacaaaatggcgaagctacacgtgcgctatatggtcggcggacgtccatcgcatccgttgcaggaacgcctctacagcttcgaattcccggaatcaccgggcgcgctgctgcgcttcctcaacacgctgggtacgtactggaacatttctttgttccactatcgcagccatggcaccgactacgggcgcgtactggcggcgttcgaacttggcgaccatgaaccggatttcgaaacccggctgaatgagctgggctacgattgccacgacgaaaccaataacccggcgttcaggttctttttggcgggttagggaaaaatgcctgatagcgcttcgcttaggcatgatgcgacgcttgttcctgcgctttgttcat

SEQ ID NO: 21 - DNA, 20 bp, Artificial Sequence
  Primer 3
aagctggtggcgtttatgca

SEQ ID NO: 22 - DNA, 20 bp, Artificial Sequence
  Primer 4
attcggcaccttccggagca

SEQ ID NO: 23 - DNA, 2131 bp, Artificial Sequence
  DNA fragment 4
aagctggtggcgtttatgcagggaatcggttttatcatcgccgggcttgccccgtggttttctggcgtgctgcgtagtatcagcggcaattacctgatggactgggcatttcatgcgctgtgcgtcgttgggctgatgatcataaccctgcgttttgcaccagtacgttttccgcagctgtgggtcaaagacgctcaagttagtataaaaaagctgaacgagaaacgtaaaatgatataaatatcaatatattaaattagattttgcataaaaaacagactacataatactgtaaaacacaacatatgcagtcactatgaatcaactacttagatggtattagtgacctgtaacagactgcagtggtcgaaaaaaaaagcccgcactgtcaggtgcgggcttttttctgtgttaagcttcgacgaatttctgccattcatccgcttattatcacttattcaggcgtagcaccaggcgtttaagggcaccaataactgccttaaaaaaattacgccccgccctgccactcatcgcagtactgttgtaattcattaagcattctgccgacatggaagccatcacagacggcatgatgaacctgaatcgccagcggcatcagcaccttgtcgccttgcgtataatatttgcccatggtgaaaacgggggcgaagaagttgtccatattggccacgtttaaatcaaaactggtgaaactcacccagggattggctgagacgaaaaacatattctcaataaaccctttagggaaataggccaggttttcaccgtaacacgccacatcttgcgaatatatgtgtagaaactgccggaaatcgtcgtggtattcactccagagcgatgaaaacgtttcagtttgctcatggaaaacggtgtaacaagggtgaacactatcccatatcaccagctcaccgtctttcattgccatacggaattccggatgagcattcatcaggcgggcaagaatgtgaataaaggccggataaaacttgtgcttatttttctttacggtctttaaaaaggccgtaatatccagctgaacggtctggttataggtacattgagcaactgactgaaatgcctcaaaatgttctttacgatgccattgggatatatcaacggtggtatatccagtgatttttttctccattttagcttccttagctcctgaaaatctcggatccgatatctagctagagcgcccggttgacgctgctagtgttacctagcgatttgtatcttactgcatgttacttcatgttgtcaatacctgtttttcgtgcgacttatcaggctgtctacttatccggagatccacaggacgggtgtggtcgccatgatcgcgtagtcgatagtggctccaagtagcgaagcgagcaggactgggcggcggccaaagcggtcggacagtgctccgagaacgggtgcgcatagaaattgcatcaacgcatatagcgctagcagcacgccatagtgactggcgatgctgtcggaatggacgatatcccgcaagaggcccggcagtaccggcataaccaagcctatgcctacagcatccagggtgacggtgccgaggatgacgatgagcgcattgttagatttcatacacggtgcctgactgcgttagcaatttaactgtgataaactaccgcattaaagcttatcgatgataagctgtcaaacatgagaattcgaaatcaaataatgattttattttgactgatagtgacctgttcgttgcaacaaattgataagcaatgcttttttataatgccaacttagtataaaaaagcaggcttcaagatcttcacctaccaaacaatgcccccctgcaaaaaataaattcatataaaaaacatacagataaccatctgcggtgataaattatctctggcggtgttgacataaataccactggcggtgatactgagcacatcagcaggacgcactgaccaccatgaaggtgacgctcttaaaaattaagccctgaagaagggcagcattcaaagcagaaggctttggggtgtgtgatacgaaacgaagcattggccggaaggagaactaactatggctgactcgcaacccctgtccggtgctccggaaggtgccgaat

SEQ ID NO: 24 - DNA, 534 bp, Artificial Sequence
  DNA fragment 5
aagctggtggcgtttatgcagggaatcggttttatcatcgccgggcttgccccgtggttttctggcgtgctgcgtagtatcagcggcaattacctgatggactgggcatttcatgcgctgtgcgtcgttgggctgatgatcataaccctgcgttttgcaccagtacgttttccgcagctgtgggtcaaagacgctcaagttagtataaaaaagcaggcttcaagatcttcacctaccaaacaatgcccccctgcaaaaaataaattcatataaaaaacatacagataaccatctgcggtgataaattatctctggcggtgttgacataaataccactggcggtgatactgagcacatcagcaggacgcactgaccaccatgaaggtgacgctcttaaaaattaagccctgaagaagggcagcattcaaagcagaaggctttggggtgtgtgatacgaaacgaagcattggccggaaggagaactaactatggctgactcgcaacccctgtccggtgctccggaaggtgccgaat

SEQ ID NO: 25 - DNA, 3195 bp, Artificial Sequence
  kdcA-aldH
ctcggtaccgaaggagggaatgtgatgtatacggtaggagattacctgttagaccgcttacacgagttgggaattgaagaaatttttggagttccgggtgactataacttacaatttttagatcaaattatttcacgcgaagatatgaaatggattggaaatgctaatgaattaaatgcttcttatatggctgatggttatgctcgtactaaaaaagctgccgcatttctcaccacgtttggagtcggcgaattgagtgcgatcaatggactggcaggaagttatgccgaaaatttaccggtagtagaaattgttggttcaccgacttcaaaagtacaaaatgacggaaaatttgtccatcatacgctggcagatggtgattttaaacactttatgaagatgcatgaaccggttacggcagcgcgcactttactgacggcagaaaatgccacgtatgaaattgaccgcgtactttctcaattactgaaagaacgcaaaccggtctatattaacttaccggtcgatgttgctgcagcaaaagcagagaagccggcattatctttagaaaaagaaagctctacgacgaatacgactgaacaagtgattttgagtaagattgaagaaagtttgaaaaatgcccaaaaaccggtagtgattgcaggacacgaagtaattagttttggtttagaaaaaacggtaactcagtttgtttcagaaacgaaactgccgattacgacgctgaattttggtaaaagtgctgttgatgaatctttgccgtcatttttaggaatttataacgggaaactttcagaaatcagtcttaaaaattttgtggagtccgcagactttatcctgatgcttggagtgaagcttacggactcctcaacgggtgcattcacgcatcatttagatgaaaataaaatgatttcactgaacattgatgaaggaattattttcaataaagtggtagaagattttgattttcgcgcagtggtttcttctttatcagaattaaaaggaattgaatatgaaggacaatatattgataagcaatatgaagaatttattccgtcaagtgctccgttatcacaagaccgtctgtggcaggcagttgaaagtttgactcaaagcaatgaaacgatcgttgctgaacaaggaacctcattttttggagcttcaacgattttcttaaaatcaaatagtcgttttattggacaaccgttatggggttctattggatatacttttccggcggctttaggaagccaaattgcggataaagagagccgccaccttttatttattggtgatggttcacttcaacttaccgtacaagaattaggactgtcaatccgcgaaaaactcaatccgatttgttttatcattaataatgatggttatacggttgaacgcgaaatccacggaccgactcaaagttataacgacattccgatgtggaattactcgaaattaccggaaacgtttggagcaacggaagatcgtgtagtatcaaaaattgttcgcacggagaatgaatttgtgtctgtcatgaaagaagcccaagcagatgtcaatcgcatgtattggattgaactggttttggaaaaagaagatgcgccgaaattactgaaaaaaatgggtaaattatttgctgagcaaaataaataaggatcctttaagaaggagatatacatatgaattttcatcatctggcttactggcaggataaagcgttaagtctcgccattgaaaaccgcttatttattaacggtgaatatactgctgcggcggaaaatgaaacctttgaaaccgttgatccggtcacccaggcaccgctggcgaaaattgcccgcggcaagagcgtcgatatcgaccgtgcgatgagcgcagcacgcggcgtatttgaacgcggcgactggtcactctcttctccggctaaacgtaaagcggtactgaataaactcgccgatttaatggaagcccacgccgaagagctggcactgctggaaactctcgacaccggcaaaccgattcgtcacagtctgcgtgatgatattcccggcgcggcgcgcgccattcgctggtacgccgaagcgatcgacaaagtgtatggcgaagtggcgaccaccagtagccatgagctggcgatgatcgtgcgtgaaccggtcggcgtgattgccgccatcgtgccgtggaacttcccgctgttgctgacttgctggaaactcggcccggcgctggcggcgggaaacagcgtgattctaaaaccgtctgaaaaatcaccgctcagtgcgattcgtctcgcggggctggcgaaagaagcaggcttgccggatggtgtgttgaacgtggtgacgggttttggtcatgaagccgggcaggcgctgtcgcgtcataacgatatcgacgccattgcctttaccggttcaacccgtaccgggaaacagctgctgaaagatgcgggcgacagcaacatgaaacgcgtctggctggaagcgggcggcaaaagcgccaacatcgttttcgctgactgcccggatttgcaacaggcggcaagcgccaccgcagcaggcattttctacaaccagggacaggtgtgcatcgccggaacgcgcctgttgctggaagagagcatcgccgatgaattcttagccctgttaaaacagcaggcgcaaaactggcagccgggccatccacttgatcccgcaaccaccatgggcaccttaatcgactgcgcccacgccgactcggtccatagctttattcgggaaggcgaaagcaaagggcaactgttgttggatggccgtaacgccgggctggctgccgccatcggcccgaccatctttgtggatgtggacccgaatgcgtccttaagtcgcgaagagattttcggtccggtgctggtggtcacgcgtttcacatcagaagaacaggcgctacagcttgccaacgacagccagtacggccttggcgcggcggtatggacgcgcgacctctcccgcgcgcaccgcatgagccgacgcctgaaagccggttccgtcttcgtcaataactacaacgacggcgatatgaccgtgccgtttggcggctataagcagagcggcaacggtcgcgacaaatccctgcatgcccttgaaaaattcactgaactgaaaaccatctggataagcctggaggcctgagatcctctagagg

SEQ ID NO: 26 - DNA, 20 bp, Artificial Sequence
  Primer P5
ctgagtaggacaaatccgcc

SEQ ID NO: 27 - DNA, 20 bp, Artificial Sequence
  Primer P6
gttatagtcacccggaactc

SEQ ID NO: 28 - DNA, 22 bp, Artificial Sequence
  Primer P7
agtagagacgaaagtgattgcg

SEQ ID NO: 29 - DNA, 20 bp, Artificial Sequence
  Primer P8
gcgacagcaacatgaaacgc

SEQ ID NO: 30 - DNA, 1045 bp, Artificial Sequence
  DNA fragment 6
ctgagtaggacaaatccgccgggagcggatttgaacgttgcgaagcaacggcccggagggtggcgggcaggacgcccgccataaactgccaggcatcaaattaagcagaaggccatcctgacggatggcctttttgcgtggctcggtaccgaaggagggaatgtgatgtatacggtaggagattacctgttagaccgcttacacgagttgggaattgaagaaatttttggagttccgggtgactataacttacaatttttagatcaaattatttcacgcgaagatatgaaatggattggaaatgctaatgaattaaatgcttcttatatggctgatggttatgctcgtactaaaaaagctgccgcatttctcaccacgtttggagtcggcgaattgagtgcgatcaatggactggcaggaagttatgccgaaaatttaccggtagtagaaattgttggttcaccgacttcaaaagtacaaaatgacggaaaatttgtccatcatacgctggcagatggtgattttaaacactttatgaagatgcatgaaccggttacggcagcgcgcactttactgacggcagaaaatgccacgtatgaaattgaccgcgtactttctcaattactgaaagaacgcaaaccggtctatattaacttaccggtcgatgttgctgcagcaaaagcagagaagccggcattatctttagaaaaagaaagctctacgacgaatacgactgaacaagtgattttgagtaagattgaagaaagtttgaaaaatgcccaaaaaccggtagtgattgcaggacacgaagtaattagttttggtttagaaaaaacggtaactcagtttgtttcagaaacgaaactgccgattacgacgctgaattttggtaaaagtgctgttgatgaatctttgccgtcatttttaggaatttataacgggaaactttcagaaatcagtcttaaaaattttgtggagtccgcagactttatcctgatgcttggagtgaagcttacggactcctcaacgggtgcattcacgcatc

SEQ ID NO: 31 - DNA, 865 bp, Artificial Sequence
  DNA fragment 7
gcgacagcaacatgaaacgcgtctggctggaagcgggcggcaaaagcgccaacatcgttttcgctgactgcccggatttgcaacaggcggcaagcgccaccgcagcaggcattttctacaaccagggacaggtgtgcatcgccggaacgcgcctgttgctggaagagagcatcgccgatgaattcttagccctgttaaaacagcaggcgcaaaactggcagccgggccatccacttgatcccgcaaccaccatgggcaccttaatcgactgcgcccacgccgactcggtccatagctttattcgggaaggcgaaagcaaagggcaactgttgttggatggccgtaacgccgggctggctgccgccatcggcccgaccatctttgtggatgtggacccgaatgcgtccttaagtcgcgaagagattttcggtccggtgctggtggtcacgcgtttcacatcagaagaacaggcgctacagcttgccaacgacagccagtacggccttggcgcggcggtatggacgcgcgacctctcccgcgcgcaccgcatgagccgacgcctgaaagccggttccgtcttcgtcaataactacaacgacggcgatatgaccgtgccgtttggcggctataagcagagcggcaacggtcgcgacaaatccctgcatgcccttgaaaaattcactgaactgaaaaccatctggataagcctggaggcctgagatcctctagaggtcgactctagaggatccccgggtaccgagctcgaattctcatgtttgacagcttatcactgatcagtgaattaatggcgatgacgcatcctcacgataatatccgggtaggcgcaatcactttcgtctctact

SEQ ID NO: 32 - DNA, 27 bp, Artificial Sequence
  Primer P9
gccatggcagaatctgctccatgcggg

SEQ ID NO: 33 - DNA, 20 bp, Artificial Sequence
  Primer P10
gttatagtcacccggaactc

SEQ ID NO: 34 - DNA, 1629 bp, Artificial Sequence
  DNA fragment 8
gccatggcagaatctgctccatgcgggacaagaaaatctcttttctggtctgacggcgcttactgctgaattcactgtcggcgaaggtaagttgatgactcatgatgaaccctgttctatggctccagatgacaaacatgatctcatatcagggacttgttcgcaccttccttagtacttcccccaataattggctggtgtttatgcaaaatggtcaagaagtggtaattgatagcggtaaaagcgttagcctcacactgacaatggctccagcttttaaggatgaaggggaactaaccgacatgacagatattacaggcaatctgacggtcctggtggaggcaaaatgaacaatgtaaaattactgattgccggaagtgccttttttgccatgtcagcgcaagccgctgatagagtatcaattgacgttaaggtgactctggaagctgcagaaaggtcatttttcctgaatatgctcacatcatataaagaaatacagataaagttattatctgcttgtggtggtgaatgcactgaccggctataaggaaaggccaaacaagacacggttgcaaaaaccgtgcccttaaatattgaatctctattcagaacactttcttaaattgtcatttggcatattacgaacaattccgcgtaaaaacgttctgttacgctaaacccttatccagcaggctttcaaggatgtaaaccataacactctgcgaactagtgttacattgcgtgtagctttgagtgggcaactttgtgtacacttttgtgtacccaaaaacaaaaatgtgtacccattcaatgatcaccgacacaaagctcaggaaggcgctcggcaagaaaagagatgatatcgagattatttctgattcgcacgagctttctagacgctcaagttagtataaaaaagctgaacgagaaacgtaaaatgatataaatatcaatatattaaattagattttgcataaaaaacagactacataatactgtaaaacacaacatatgcagtcactatgaatcaactacttagatggtattagtgacctgtaacagactgcgggcccaggttatgctgcttttaagacccactttcacatttaagttgtttttctaatccgcatatgatcaattcaaggccgaataagaaggctggctctgcaccttggtgatcaaataattcgatagcttgtcgtaataatggcggcatactatcagtagtaggtgtttccctttcttctttagcgacttgatgctcttgatcttccaatacgcaacctaaagtaaaatgccccacagcgctgagtgcatataatgcattctctagtgaaaaaccttgttggcataaaaaggctaattgattttcgagagtttcatactgtttttctgtaggccgtgtacctaaatgtacttttgctccatcgcgatgacttagtaaagcacatctaaaacttttagcgttattacgtaaaaaatcttgccagctttccccttctaaagggcaaaagtgagtatggtgcctatctaacatctcaatggctaaggcgtcgagcaaagcccgcttattttttacatgccaatacaatgtaggctgctctacacctagcttctgggcgagtttac

SEQ ID NO: 35 - DNA, 22 bp, Artificial Sequence
  Primer P11
gtaaactcgcccagaagctagg

SEQ ID NO: 36 - DNA, 4603 bp, Artificial Sequence
  DNA fragment 9
gccatggcagaatctgctccatgcgggacaagaaaatctcttttctggtctgacggcgcttactgctgaattcactgtcggcgaaggtaagttgatgactcatgatgaaccctgttctatggctccagatgacaaacatgatctcatatcagggacttgttcgcaccttccttagtacttcccccaataattggctggtgtttatgcaaaatggtcaagaagtggtaattgatagcggtaaaagcgttagcctcacactgacaatggctccagcttttaaggatgaaggggaactaaccgacatgacagatattacaggcaatctgacggtcctggtggaggcaaaatgaacaatgtaaaattactgattgccggaagtgccttttttgccatgtcagcgcaagccgctgatagagtatcaattgacgttaaggtgactctggaagctgcagaaaggtcatttttcctgaatatgctcacatcatataaagaaatacagataaagttattatctgcttgtggtggtgaatgcactgaccggctataaggaaaggccaaacaagacacggttgcaaaaaccgtgcccttaaatattgaatctctattcagaacactttcttaaattgtcatttggcatattacgaacaattccgcgtaaaaacgttctgttacgctaaacccttatccagcaggctttcaaggatgtaaaccataacactctgcgaactagtgttacattgcgtgtagctttgagtgggcaactttgtgtacacttttgtgtacccaaaaacaaaaatgtgtacccattcaatgatcaccgacacaaagctcaggaaggcgctcggcaagaaaagagatgatatcgagattatttctgattcgcacgagctttctagacgctcaagttagtataaaaaagctgaacgagaaacgtaaaatgatataaatatcaatatattaaattagattttgcataaaaaacagactacataatactgtaaaacacaacatatgcagtcactatgaatcaactacttagatggtattagtgacctgtaacagactgcgggcccaggttatgctgcttttaagacccactttcacatttaagttgtttttctaatccgcatatgatcaattcaaggccgaataagaaggctggctctgcaccttggtgatcaaataattcgatagcttgtcgtaataatggcggcatactatcagtagtaggtgtttccctttcttctttagcgacttgatgctcttgatcttccaatacgcaacctaaagtaaaatgccccacagcgctgagtgcatataatgcattctctagtgaaaaaccttgttggcataaaaaggctaattgattttcgagagtttcatactgtttttctgtaggccgtgtacctaaatgtacttttgctccatcgcgatgacttagtaaagcacatctaaaacttttagcgttattacgtaaaaaatcttgccagctttccccttctaaagggcaaaagtgagtatggtgcctatctaacatctcaatggctaaggcgtcgagcaaagcccgcttattttttacatgccaatacaatgtaggctgctctacacctagcttctgggcgagtttacgggttgttaaaccttcgattccgacctcattaagcagctctaatgcgctgttaatcactttacttttatctaatctagacatcattaattcctaatttttgttgacactctatcattgatagagttattttaccactccctatcagtgatagagaaaagtgaaatgaatagttcgacaaagatcgcattggtaattacgttactcgatgccatggggattggccttatcatgccagtcttgccaacgttattacgtgaatttattgcttcggaagatatcgctaaccactttggcgtattgcttgcactttatgcgttaatgcaggttatctttgctccttggcttggaaaaatgtctgaccgatttggtcggcgcccagtgctgttgttgtcattaataggcgcatcgctggattacttattgctggctttttcaagtgcgctttggatgctgtatttaggccgtttgctttcagggatcacaggagctactggggctgtcgcggcatcggtcattgccgataccacctcagcttctcaacgcgtgaagtggttcggttggttaggggcaagttttgggcttggtttaatagcggggcctattattggtggttttgcaggagagatttcaccgcatagtcccttttttatcgctgcgttgctaaatattgtcactttccttgtggttatgttttggttccgtgaaaccaaaaatacacgtgataatacagataccgaagtaggggttgagacgcaatcgaattcggtatacatcactttatttaaaacgatgcccattttgttgattatttatttttcagcgcaattgataggccaaattcccgcaacggtgtgggtgctatttaccgaaaatcgttttggatggaatagcatgatggttggcttttcattagcgggtcttggtcttttacactcagtattccaagcctttgtggcaggaagaatagccactaaatggggcgaaaaaacggcagtactgctcgaatttattgcagatagtagtgcatttgcctttttagcgtttatatctgaaggttggttagatttccctgttttaattttattggctggtggtgggatcgctttacctgcattacagggagtgatgtctatccaaacaaagagtcatgagcaaggtgctttacagggattattggtgagccttaccaatgcaaccggtgttattggcccattactgtttactgttatttataatcattcactaccaatttgggatggctggatttggattattggtttagcgttttactgtattattatcctgctatcgatgaccttcatgttaacccctcaagctcaggggagtaaacaggagacaagtgcttagttatttcgtcaccaaatgatgttattccgcgaaatataatgaccctcttgataacccaagagggcattttttacgagacgtcctaattcccatgtcagccgttaagtgttcctgtgtcactgaaaattgctttgagaggctctaagggcttctcagtgcgttacatccctggcttgttgtccacaaccgttaaaccttaaaagctttaaaagccttatatattcttttttttcttataaaacttaaaaccttagaggctatttaagttgctgatttatattaattttattgttcaaacatgagagcttagtacgtgaaacatgagagcttagtacgttagccatgagagcttagtacgttagccatgagggtttagttcgttaaacatgagagcttagtacgttaaacatgagagcttagtacgtgaaacatgagagcttagtacgtactatcaacaggttgaactgctgatcttcagatcctctacgccggacgcatcgtggccggatcttgcggccgcaaaaattaaaaatgaagttttggaggcctcatttggtgacgaaataactaagcacttgtctcctgtttactcccctgagcttgaggggtcaacatgaaggtcattgatagcaggataataatacagtaaaacgctaaaccaataatccaaatccagccatcccaaattggtagtgaatgattataaataacagtaaacagtaatgggccaataacaccggttgcattggtaaggctcaccaataatccctgtaaagcaccttgctcatgactctttgtttggatagacatcactccctgtaatgcaggtaaagcgatcccaccaccagccaataaaattaaaacagggaaatctaaccaaccttcagatataaacgctaaaaaggcaaatgcactactatctgcaataaattcgagcagtactgccgttttttcgccccatttagtggctattcttcctgccacaaaggcttggaatactgagtgtaaaagaccaagacccgctaatgaaaagccaaccatcatgctattccatccaaaacgattttcggtaaatagcacccacaccgttgcgggaatttggcctatcaattcgaaatcaaataatgattttattttgactgatagtgacctgttcgttgcaacaaattgataagcaatgcttttttataatgccaacttagtataaaaaagcaggcttcagagcgatggcccccgatggtagtgtggggtctccccatgcgagagtagggaactgccaggcatcaaataaaacgaaaggctcagtcgaaagactgggcctttcgttttatctgttgtttgtcggtgaacgctctcctgagtaggacaaatccgccgggagcggatttgaacgttgcgaagcaacggcccggagggtggcgggcaggacgcccgccataaactgccaggcatcaaattaagcagaaggccatcctgacggatggcctttttgcgtggctcggtaccgaaggagggaatgtgatgtatacggtaggagattacctgttagaccgcttacacgagttgggaattgaagaaatttttggagttccgggtgactataac

SEQ ID NO: 37 - DNA, 1312 bp, Artificial Sequence
  DNA fragment 10
gccatggcagaatctgctccatgcgggacaagaaaatctcttttctggtctgacggcgcttactgctgaattcactgtcggcgaaggtaagttgatgactcatgatgaaccctgttctatggctccagatgacaaacatgatctcatatcagggacttgttcgcaccttccttagtacttcccccaataattggctggtgtttatgcaaaatggtcaagaagtggtaattgatagcggtaaaagcgttagcctcacactgacaatggctccagcttttaaggatgaaggggaactaaccgacatgacagatattacaggcaatctgacggtcctggtggaggcaaaatgaacaatgtaaaattactgattgccggaagtgccttttttgccatgtcagcgcaagccgctgatagagtatcaattgacgttaaggtgactctggaagctgcagaaaggtcatttttcctgaatatgctcacatcatataaagaaatacagataaagttattatctgcttgtggtggtgaatgcactgaccggctataaggaaaggccaaacaagacacggttgcaaaaaccgtgcccttaaatattgaatctctattcagaacactttcttaaattgtcatttggcatattacgaacaattccgcgtaaaaacgttctgttacgctaaacccttatccagcaggctttcaaggatgtaaaccataacactctgcgaactagtgttacattgcgtgtagctttgagtgggcaactttgtgtacacttttgtgtacccaaaaacaaaaatgtgtacccattcaatgatcaccgacacaaagctcaggaaggcgctcggcaagaaaagagatgatatcgagattatttctgattcgcacgagctttctagacgctcaagttagtataaaaaagcaggcttcagagcgatggcccccgatggtagtgtggggtctccccatgcgagagtagggaactgccaggcatcaaataaaacgaaaggctcagtcgaaagactgggcctttcgttttatctgttgtttgtcggtgaacgctctcctgagtaggacaaatccgccgggagcggatttgaacgttgcgaagcaacggcccggagggtggcgggcaggacgcccgccataaactgccaggcatcaaattaagcagaaggccatcctgacggatggcctttttgcgtggctcggtaccgaaggagggaatgtgatgtatacggtaggagattacctgttagaccgcttacacgagttgggaattgaagaaatttttggagttccgggtgactataac

SEQ ID NO: 38 - DNA, 64 bp, Artificial Sequence
  Primer P12
gtagtgtggggtctccccatgcgagagtagggaactcgctcaagttagtataaaaaagctgaac

SEQ ID NO: 39 - DNA, 64 bp, Artificial Sequence
  Primer P13
gtaatctcctaccgtatacatcacattccctccttcgctcacaattccacacattatacgagcc

SEQ ID NO: 40 - DNA, 1768 bp, Artificial Sequence
  DNA fragment 11
gtagtgtggggtctccccatgcgagagtagggaactcgctcaagttagtataaaaaagctgaacgagaaacgtaaaatgatataaatatcaatatattaaattagattttgcataaaaaacagactacataatactgtaaaacacaacatatgcagtcactatgaatcaactacttagatggtattagtgacctgtaacagactgcagtggtcgaaaaaaaaagcccgcactgtcaggtgcgggcttttttctgtgttaagcttcgacgaatttctgccattcatccgcttattatcacttattcaggcgtagcaccaggcgtttaagggcaccaataactgccttaaaaaaattacgccccgccctgccactcatcgcagtactgttgtaattcattaagcattctgccgacatggaagccatcacagacggcatgatgaacctgaatcgccagcggcatcagcaccttgtcgccttgcgtataatatttgcccatggtgaaaacgggggcgaagaagttgtccatattggccacgtttaaatcaaaactggtgaaactcacccagggattggctgagacgaaaaacatattctcaataaaccctttagggaaataggccaggttttcaccgtaacacgccacatcttgcgaatatatgtgtagaaactgccggaaatcgtcgtggtattcactccagagcgatgaaaacgtttcagtttgctcatggaaaacggtgtaacaagggtgaacactatcccatatcaccagctcaccgtctttcattgccatacggaattccggatgagcattcatcaggcgggcaagaatgtgaataaaggccggataaaacttgtgcttatttttctttacggtctttaaaaaggccgtaatatccagctgaacggtctggttataggtacattgagcaactgactgaaatgcctcaaaatgttctttacgatgccattgggatatatcaacggtggtatatccagtgatttttttctccattttagcttccttagctcctgaaaatctcggatccggccaagctagcttggctctagctagagcgcccggttgacgctgctagtgttacctagcgatttgtatcttactgcatgttacttcatgttgtcaatacctgtttttcgtgcgacttatcaggctgtctacttatccggagatccacaggacgggtgtggtcgccatgatcgcgtagtcgatagtggctccaagtagcgaagcgagcaggactgggcggcggccaaagcggtcggacagtgctccgagaacgggtgcgcatagaaattgcatcaacgcatatagcgctagcagcacgccatagtgactggcgatgctgtcggaatggacgatatcccgcaagaggcccggcagtaccggcataaccaagcctatgcctacagcatccagggtgacggtgccgaggatgacgatgagcgcattgttagatttcatacacggtgcctgactgcgttagcaatttaactgtgataaactaccgcattaaagcttatcgatgataagctgtcaaacatgagaattcgaaatcaaataatgattttattttgactgatagtgacctgttcgttgcaacaaattgataagcaatgcttttttataatgccaacttagtataaaaaagcaggcttcaagatctccctgttgacaattaatcatcggctcgtataatgtgtggaattgtgagcgaaggagggaatgtgatgtatacggtaggagattac

SEQ ID NO: 41 - DNA, 20 bp, Artificial Sequence
  Primer P14
gatagtgacctgttcgttgc

SEQ ID NO: 42 - DNA, 1030 bp, Artificial Sequence
  DNA fragment 12
gatagtgacctgttcgttgcaacaaattgataagcaatgcttttttataatgccaacttagtataaaaaagcaggcttcaagatctccctgttgacaattaatcatcggctcgtataatgtgtggaattgtgagcgaaggagggaatgtgatgtatacggtaggagattacctgttagaccgcttacacgagttgggaattgaagaaatttttggagttccgggtgactataacttacaatttttagatcaaattatttcacgcgaagatatgaaatggattggaaatgctaatgaattaaatgcttcttatatggctgatggttatgctcgtactaaaaaagctgccgcatttctcaccacgtttggagtcggcgaattgagtgcgatcaatggactggcaggaagttatgccgaaaatttaccggtagtagaaattgttggttcaccgacttcaaaagtacaaaatgacggaaaatttgtccatcatacgctggcagatggtgattttaaacactttatgaagatgcatgaaccggttacggcagcgcgcactttactgacggcagaaaatgccacgtatgaaattgaccgcgtactttctcaattactgaaagaacgcaaaccggtctatattaacttaccggtcgatgttgctgcagcaaaagcagagaagccggcattatctttagaaaaagaaagctctacgacgaatacgactgaacaagtgattttgagtaagattgaagaaagtttgaaaaatgcccaaaaaccggtagtgattgcaggacacgaagtaattagttttggtttagaaaaaacggtaactcagtttgtttcagaaacgaaactgccgattacgacgctgaattttggtaaaagtgctgttgatgaatctttgccgtcatttttaggaatttataacgggaaactttcagaaatcagtcttaaaaattttgtggagtccgcagactttatcctgatgcttggagtgaagcttacggactcctcaacgggtgcattcacgcatc

SEQ ID NO: 43 - DNA, 20 bp, Artificial Sequence
  Primer P15
gccatggcagaatctgctcc

SEQ ID NO: 44 - DNA, 2777 bp, Artificial Sequence
  DNA fragment 13
gccatggcagaatctgctccatgcgggacaagaaaatctcttttctggtctgacggcgcttactgctgaattcactgtcggcgaaggtaagttgatgactcatgatgaaccctgttctatggctccagatgacaaacatgatctcatatcagggacttgttcgcaccttccttagtacttcccccaataattggctggtgtttatgcaaaatggtcaagaagtggtaattgatagcggtaaaagcgttagcctcacactgacaatggctccagcttttaaggatgaaggggaactaaccgacatgacagatattacaggcaatctgacggtcctggtggaggcaaaatgaacaatgtaaaattactgattgccggaagtgccttttttgccatgtcagcgcaagccgctgatagagtatcaattgacgttaaggtgactctggaagctgcagaaaggtcatttttcctgaatatgctcacatcatataaagaaatacagataaagttattatctgcttgtggtggtgaatgcactgaccggctataaggaaaggccaaacaagacacggttgcaaaaaccgtgcccttaaatattgaatctctattcagaacactttcttaaattgtcatttggcatattacgaacaattccgcgtaaaaacgttctgttacgctaaacccttatccagcaggctttcaaggatgtaaaccataacactctgcgaactagtgttacattgcgtgtagctttgagtgggcaactttgtgtacacttttgtgtacccaaaaacaaaaatgtgtacccattcaatgatcaccgacacaaagctcaggaaggcgctcggcaagaaaagagatgatatcgagattatttctgattcgcacgagctttctagacgctcaagttagtataaaaaagcaggcttcagagcgatggcccccgatggtagtgtggggtctccccatgcgagagtagggaactcgctcaagttagtataaaaaagctgaacgagaaacgtaaaatgatataaatatcaatatattaaattagattttgcataaaaaacagactacataatactgtaaaacacaacatatgcagtcactatgaatcaactacttagatggtattagtgacctgtaacagactgcagtggtcgaaaaaaaaagcccgcactgtcaggtgcgggcttttttctgtgttaagcttcgacgaatttctgccattcatccgcttattatcacttattcaggcgtagcaccaggcgtttaagggcaccaataactgccttaaaaaaattacgccccgccctgccactcatcgcagtactgttgtaattcattaagcattctgccgacatggaagccatcacagacggcatgatgaacctgaatcgccagcggcatcagcaccttgtcgccttgcgtataatatttgcccatggtgaaaacgggggcgaagaagttgtccatattggccacgtttaaatcaaaactggtgaaactcacccagggattggctgagacgaaaaacatattctcaataaaccctttagggaaataggccaggttttcaccgtaacacgccacatcttgcgaatatatgtgtagaaactgccggaaatcgtcgtggtattcactccagagcgatgaaaacgtttcagtttgctcatggaaaacggtgtaacaagggtgaacactatcccatatcaccagctcaccgtctttcattgccatacggaattccggatgagcattcatcaggcgggcaagaatgtgaataaaggccggataaaacttgtgcttatttttctttacggtctttaaaaaggccgtaatatccagctgaacggtctggttataggtacattgagcaactgactgaaatgcctcaaaatgttctttacgatgccattgggatatatcaacggtggtatatccagtgatttttttctccattttagcttccttagctcctgaaaatctcggatccggccaagctagcttggctctagctagagcgcccggttgacgctgctagtgttacctagcgatttgtatcttactgcatgttacttcatgttgtcaatacctgtttttcgtgcgacttatcaggctgtctacttatccggagatccacaggacgggtgtggtcgccatgatcgcgtagtcgatagtggctccaagtagcgaagcgagcaggactgggcggcggccaaagcggtcggacagtgctccgagaacgggtgcgcatagaaattgcatcaacgcatatagcgctagcagcacgccatagtgactggcgatgctgtcggaatggacgatatcccgcaagaggcccggcagtaccggcataaccaagcctatgcctacagcatccagggtgacggtgccgaggatgacgatgagcgcattgttagatttcatacacggtgcctgactgcgttagcaatttaactgtgataaactaccgcattaaagcttatcgatgataagctgtcaaacatgagaattcgaaatcaaataatgattttattttgactgatagtgacctgttcgttgcaacaaattgataagcaatgcttttttataatgccaacttagtataaaaaagcaggcttcaagatctccctgttgacaattaatcatcggctcgtataatgtgtggaattgtgagcgaaggagggaatgtgatgtatacggtaggagattacctgttagaccgcttacacgagttgggaattgaagaaatttttggagttccgggtgactataac

SEQ ID NO: 45 - DNA, 1167 bp, Artificial Sequence
  DNA fragment 14
gccatggcagaatctgctccatgcgggacaagaaaatctcttttctggtctgacggcgcttactgctgaattcactgtcggcgaaggtaagttgatgactcatgatgaaccctgttctatggctccagatgacaaacatgatctcatatcagggacttgttcgcaccttccttagtacttcccccaataattggctggtgtttatgcaaaatggtcaagaagtggtaattgatagcggtaaaagcgttagcctcacactgacaatggctccagcttttaaggatgaaggggaactaaccgacatgacagatattacaggcaatctgacggtcctggtggaggcaaaatgaacaatgtaaaattactgattgccggaagtgccttttttgccatgtcagcgcaagccgctgatagagtatcaattgacgttaaggtgactctggaagctgcagaaaggtcatttttcctgaatatgctcacatcatataaagaaatacagataaagttattatctgcttgtggtggtgaatgcactgaccggctataaggaaaggccaaacaagacacggttgcaaaaaccgtgcccttaaatattgaatctctattcagaacactttcttaaattgtcatttggcatattacgaacaattccgcgtaaaaacgttctgttacgctaaacccttatccagcaggctttcaaggatgtaaaccataacactctgcgaactagtgttacattgcgtgtagctttgagtgggcaactttgtgtacacttttgtgtacccaaaaacaaaaatgtgtacccattcaatgatcaccgacacaaagctcaggaaggcgctcggcaagaaaagagatgatatcgagattatttctgattcgcacgagctttctagacgctcaagttagtataaaaaagcaggcttcagagcgatggcccccgatggtagtgtggggtctccccatgcgagagtagggaactcgctcaagttagtataaaaaagcaggcttcaagatctccctgttgacaattaatcatcggctcgtataatgtgtggaattgtgagcgaaggagggaatgtgatgtatacggtaggagattacctgttagaccgcttacacgagttgggaattgaagaaatttttggagttccgggtgactataac

SEQ ID NO: 46 - DNA, 64 bp, Artificial Sequence
  Primer P16
cagagcacaaccacatcacaacaaatccgcgcctgatgaagcctgcttttttatactaagttgg

SEQ ID NO: 47 - DNA, 64 bp, Artificial Sequence
  Primer P17
catactttatttactcccagtgtctgtctcgtaaatcgctcaagttagtataaaaaagctgaac

SEQ ID NO: 48 - DNA, 1713 bp, Artificial Sequence
  DNA fragment 15
cagagcacaacctcatcacaacaaatccgcgcctgatgaagcctgcttttttatactaagttggcattataaaaaagcattgcttatcaatttgttgcaacgaacaggtcactatcagtcaaaataaaatcattatttgatttcgaattctcatgtttgacagcttatcatcgataagctttaatgcggtagtttatcacagttaaattgctaacgcagtcaggcaccgtgtatgaaatctaacaatgcgctcatcgtcatcctcggcaccgtcaccctggatgctgtaggcataggcttggttatgccggtactgccgggcctcttgcgggatatcgtccattccgacagcatcgccagtcactatggcgtgctgctagcgctatatgcgttgatgcaatttctatgcgcacccgttctcggagcactgtccgaccgctttggccgccgcccagtcctgctcgcttcgctacttggagccactatcgactacgcgatcatggcgaccacacccgtcctgtggatctccggataagtagacagcctgataagtcgcacgaaaaacaggtattgacaacatgaagtaacatgcagtaagatacaaatcgctaggtaacactagcagcgtcaaccgggcgctctagctagagccaagctagcttggccggatccgagattttcaggagctaaggaagctaaaatggagaaaaaaatcactggatataccaccgttgatatatcccaatggcatcgtaaagaacattttgaggcatttcagtcagttgctcaatgtacctataaccagaccgttcagctggatattacggcctttttaaagaccgtaaagaaaaataagcacaagttttatccggcctttattcacattcttgcccgcctgatgaatgctcatccggaattccgtatggcaatgaaagacggtgagctggtgatatgggatagtgttcacccttgttacaccgttttccatgagcaaactgaaacgttttcatcgctctggagtgaataccacgacgatttccggcagtttctacacatatattcgcaagatgtggcgtgttacggtgaaaacctggcctatttccctaaagggtttattgagaatatgtttttcgtctcagccaatccctgggtgagtttcaccagttttgatttaaacgtggccaatatggacaacttcttcgcccccgttttcaccatgggcaaatattatacgcaaggcgacaaggtgctgatgccgctggcgattcaggttcatcatgccgtctgtgatggcttccatgtcggcagaatgcttaatgaattacaacagtactgcgatgagtggcagggcggggcgtaatttttttaaggcagttattggtgcccttaaacgcctggtgctacgcctgaataagtgataataagcggatgaatggcagaaattcgtcgaagcttaacacagaaaaaagcccgcacctgacagtgcgggctttttttttcgaccactgcagtctgttacaggtcactaataccatctaagtagttgattcatagtgactgcatatgttgtgttttacagtattatgtagtctgttttttatgcaaaatctaatttaatatattgatatttatatcattttacgtttctcgttcagcttttttatactaacttgagcgatttacgagacagacactgggagtaaataaagtatg

SEQ ID NO: 49 - DNA, 21 bp, Artificial Sequence
  Primer P18
ccagtaattcagaaatgttgg

SEQ ID NO: 50 - DNA, 21 bp, Artificial Sequence
  Primer P19
ccatattacgaccatgagtgg

SEQ ID NO: 51 - DNA, 1354 bp, Artificial Sequence
  DNA fragment 16
ccagtaattcagaaatgttggagaaattatcatgatgcaacatcaggtcaatgtatcggctcgcttcaatccagaaaccttagaacgtgttttacgcgtggtgcgtcatcgtggtttccacgtctgctcaatgaatatggccgccgccagcgatgcacaaaatataaatatcgaattgaccgttgccagcccacggtcggtcgacttactgtttagtcagttaaataaactggtggacgtcgcacacgttgccatctgccagagcacaaccacatcacaacaaatccgcgcctgagcgcaaaaggaatataaaaatgaccacgaagaaagctgattacatttggttcaatggggagatggttcgctgggaagacgcgaaggtgcatgtgatgtcgcacgcgctgcactatggcacttcggtttttgaaggcatccgttgctacgactcgcacaaaggaccggttgtattccgccatcgtgagcatatgcagcgtctgcatgactccgccaaaatctatcgcttcccggtttcgcagagcattgatgagctgatggaagcttgtcgtgacgtgatccgcaaaaacaatctcaccagcgcctatatccgtccgctgatcttcgtcggtgatgttggcatgggagtaaacccgccagcgggatactcaaccgacgtgattatcgctgctttcccgtggggagcgtatctgggcgcagaagcgctggagcaggggatcgatgcgatggtttcctcctggaaccgcgcacgaccaaacaccatcccgacggcggcaaaagccggtggtaactacctctcttccctgctggtgggtagcgaagcgcgccgccacggttatcaggaaggtatcgcgctggatgtgaacggttatatctctgaaggcgcaggcgaaaacctgtttgaagtgaaagatggtgtgctgttcaccccaccgttcacctcctccgcgctgccgggtattacccgtgatgccatcatcaaactggcgaaagagctgggaattgaagtacgtgagcaggtgctgtcgcgcgaatccctgtacctggcggatgaagtgtttatgtccggtacggcggcagaaatcacgccagtgcgcagcgtagacggtattcaggttggcgaaggccgttgtggcccggttaccaaacgcattcagcaagccttcttcggcctcttcactggcgaaaccgaagataaatggggctggttagatcaagttaatcaataaatacaaaaaatgggacggcacgcaccgtcccatttacgagacagacactgggagtaaataaagtatgcctaagtaccgttccgccaccaccactcatggtcgtaatatgg

SEQ ID NO: 52 - DNA, 2015 bp, Artificial Sequence
  DNA fragment 17
ccagtaattcagaaatgttggagaaattatcatgatgcaacatcaggtcaatgtatcggctcgcttcaatccagaaaccttagaacgtgttttacgcgtggtgcgtcatcgtggtttccacgtctgctcaatgaatatggccgccgccagcgatgcacaaaatataaatatcgaattgaccgttgccagcccacggtcggtcgacttactgtttagtcagttaaataaactggtggacgtcgcacacgttgccatctgccagagcacaacctcatcacaacaaatccgcgcctgatgaagcctgcttttttatactaagttggcattataaaaaagcattgcttatcaatttgttgcaacgaacaggtcactatcagtcaaaataaaatcattatttgatttcgaattctcatgtttgacagcttatcatcgataagctttaatgcggtagtttatcacagttaaattgctaacgcagtcaggcaccgtgtatgaaatctaacaatgcgctcatcgtcatcctcggcaccgtcaccctggatgctgtaggcataggcttggttatgccggtactgccgggcctcttgcgggatatcgtccattccgacagcatcgccagtcactatggcgtgctgctagcgctatatgcgttgatgcaatttctatgcgcacccgttctcggagcactgtccgaccgctttggccgccgcccagtcctgctcgcttcgctacttggagccactatcgactacgcgatcatggcgaccacacccgtcctgtggatctccggataagtagacagcctgataagtcgcacgaaaaacaggtattgacaacatgaagtaacatgcagtaagatacaaatcgctaggtaacactagcagcgtcaaccgggcgctctagctagagccaagctagcttggccggatccgagattttcaggagctaaggaagctaaaatggagaaaaaaatcactggatataccaccgttgatatatcccaatggcatcgtaaagaacattttgaggcatttcagtcagttgctcaatgtacctataaccagaccgttcagctggatattacggcctttttaaagaccgtaaagaaaaataagcacaagttttatccggcctttattcacattcttgcccgcctgatgaatgctcatccggaattccgtatggcaatgaaagacggtgagctggtgatatgggatagtgttcacccttgttacaccgttttccatgagcaaactgaaacgttttcatcgctctggagtgaataccacgacgatttccggcagtttctacacatatattcgcaagatgtggcgtgttacggtgaaaacctggcctatttccctaaagggtttattgagaatatgtttttcgtctcagccaatccctgggtgagtttcaccagttttgatttaaacgtggccaatatggacaacttcttcgcccccgttttcaccatgggcaaatattatacgcaaggcgacaaggtgctgatgccgctggcgattcaggttcatcatgccgtctgtgatggcttccatgtcggcagaatgcttaatgaattacaacagtactgcgatgagtggcagggcggggcgtaatttttttaaggcagttattggtgcccttaaacgcctggtgctacgcctgaataagtgataataagcggatgaatggcagaaattcgtcgaagcttaacacagaaaaaagcccgcacctgacagtgcgggctttttttttcgaccactgcagtctgttacaggtcactaataccatctaagtagttgattcatagtgactgcatatgttgtgttttacagtattatgtagtctgttttttatgcaaaatctaatttaatatattgatatttatatcattttacgtttctcgttcagcttttttatactaacttgagcgatttacgagacagacactgggagtaaataaagtatgcctaagtaccgttccgccaccaccactcatggtcgtaatatgg

SEQ ID NO: 53 - DNA, 405 bp, Artificial Sequence
  DNA fragment 18
ccagtaattcagaaatgttggagaaattatcatgatgcaacatcaggtcaatgtatcggctcgcttcaatccagaaaccttagaacgtgttttacgcgtggtgcgtcatcgtggtttccacgtctgctcaatgaatatggccgccgccagcgatgcacaaaatataaatatcgaattgaccgttgccagcccacggtcggtcgacttactgtttagtcagttaaataaactggtggacgtcgcacacgttgccatctgccagagcacaaccacatcacaacaaatccgcgcctgatgaagcctgcttttttatactaacttgagcgatttacgagacagacactgggagtaaataaagtatgcctaagtaccgttccgccaccaccactcatggtcgtaatatgg

SEQ ID NO: 54 - DNA, 64 bp, Artificial Sequence
  Primer P20
aaccacctgcccgtaaacctggagaaccatcgcgtgtgaagcctgcttttttatactaagttgg

SEQ ID NO: 55 - DNA, 64 bp, Artificial Sequence
  Primer P21
agctccagcctgctttcctgcattacatcaccgcagcgctcaagttagtataaaaaagctgaac

SEQ ID NO: 56 - DNA, 1713 bp, Artificial Sequence
  DNA fragment 19
aaccacctgcccgtaaacctggagaaccatcgcgtgtgaagcctgcttttttatactaagttggcattataaaaaagcattgcttatcaatttgttgcaacgaacaggtcactatcagtcaaaataaaatcattatttgatttcgaattctcatgtttgacagcttatcatcgataagctttaatgcggtagtttatcacagttaaattgctaacgcagtcaggcaccgtgtatgaaatctaacaatgcgctcatcgtcatcctcggcaccgtcaccctggatgctgtaggcataggcttggttatgccggtactgccgggcctcttgcgggatatcgtccattccgacagcatcgccagtcactatggcgtgctgctagcgctatatgcgttgatgcaatttctatgcgcacccgttctcggagcactgtccgaccgctttggccgccgcccagtcctgctcgcttcgctacttggagccactatcgactacgcgatcatggcgaccacacccgtcctgtggatctccggataagtagacagcctgataagtcgcacgaaaaacaggtattgacaacatgaagtaacatgcagtaagatacaaatcgctaggtaacactagcagcgtcaaccgggcgctctagctagagccaagctagcttggccggatccgagattttcaggagctaaggaagctaaaatggagaaaaaaatcactggatataccaccgttgatatatcccaatggcatcgtaaagaacattttgaggcatttcagtcagttgctcaatgtacctataaccagaccgttcagctggatattacggcctttttaaagaccgtaaagaaaaataagcacaagttttatccggcctttattcacattcttgcccgcctgatgaatgctcatccggaattccgtatggcaatgaaagacggtgagctggtgatatgggatagtgttcacccttgttacaccgttttccatgagcaaactgaaacgttttcatcgctctggagtgaataccacgacgatttccggcagtttctacacatatattcgcaagatgtggcgtgttacggtgaaaacctggcctatttccctaaagggtttattgagaatatgtttttcgtctcagccaatccctgggtgagtttcaccagttttgatttaaacgtggccaatatggacaacttcttcgcccccgttttcaccatgggcaaatattatacgcaaggcgacaaggtgctgatgccgctggcgattcaggttcatcatgccgtctgtgatggcttccatgtcggcagaatgcttaatgaattacaacagtactgcgatgagtggcagggcggggcgtaatttttttaaggcagttattggtgcccttaaacgcctggtgctacgcctgaataagtgataataagcggatgaatggcagaaattcgtcgaagcttaacacagaaaaaagcccgcacctgacagtgcgggctttttttttcgaccactgcagtctgttacaggtcactaataccatctaagtagttgattcatagtgactgcatatgttgtgttttacagtattatgtagtctgttttttatgcaaaatctaatttaatatattgatatttatatcattttacgtttctcgttcagcttttttatactaacttgagcgctgcggtgatgtaatgcaggaaagcaggctggagct

SEQ ID NO: 57 - DNA, 21 bp, Artificial Sequence
  Primer P22
ggatgtacgtttgtcatgagt

SEQ ID NO: 58 - DNA, 20 bp, Artificial Sequence
  Primer P23
tctcacgtagaacgatggca

SEQ ID NO: 59 - DNA, 1430 bp, Artificial Sequence
  DNA fragment 20
ggatgtacgtttgtcatgagtctcactctgttgctaattgccgttcgctcctgaacatccactcgatcttcgccttcttccggtttattgtgttttaaccacctgcccgtaaacctggagaaccatcgcgtgtttcaaaaagttgacgcctacgctggcgacccgattcttacgcttatggagcgttttaaagaagaccctcgcagcgacaaagtgaatttaagtatcggtctgtactacaacgaagacggaattattccacaactgcaagccgtggcggaggcggaagcgcgcctgaatgcgcagcctcatggcgcttcgctttatttaccgatggaagggcttaactgctatcgccatgccattgcgccgctgctgtttggtgcggaccatccggtactgaaacaacagcgcgtagcaaccattcaaacccttggcggctccggggcattgaaagtgggcgcggatttcctgaaacgctacttcccggaatcaggcgtctgggtcagcgatcctacctgggaaaaccacgtagcaatattcgccggggctggattcgaagtgagtacttacccctggtatgacgaagcgactaacggcgtgcgctttaatgacctgttggcgacgctgaaaacattacctgcccgcagtattgtgttgctgcatccatgttgccacaacccaacgggtgccgatctcactaatgatcagtgggatgcggtgattgaaattctcaaagcccgcgagcttattccattcctcgatattgcctatcaaggatttggtgccggtatggaagaggatgcctacgctattcgcgccattgccagcgctggattacccgctctggtgagcaattcgttctcgaaaattttctccctttacggcgagcgcgtcggcggactttctgttatgtgtgaagatgccgaagccgctggccgcgtactggggcaattgaaagcaacagttcgccgcaactactccagcccgccgaattttggtgcgcaggtggtggctgcagtgctgaatgacgaggcattgaaagccagctggctggcggaagtagaagagatgcgtactcgcattctggcaatgcgtcaggaattggtgaaggtattaagcacagagatgccagaacgcaatttcgattatctgcttaatcagcgcggcatgttcagttataccggtttaagtgccgctcaggttgaccgactacgtgaagaatttggtgtctatctcatcgccagcggtcgcatgtgtgtcgccgggttaaatacggcaaatgtacaacgtgtggcaaaggcgtttgctgcggtgatgtaatgcaggaaagcaggctggagctacccagcctgcagtgaaattaaactgtcgtcgctttcactctttctttatagatgatttttttgatgccatcgttctacgtgaga

SEQ ID NO: 60 - DNA, 1894 bp, Artificial Sequence
  DNA fragment 21
ggatgtacgtttgtcatgagtctcactctgttgctaattgccgttcgctcctgaacatccactcgatcttcgccttcttccggtttattgtgttttaaccacctgcccgtaaacctggagaaccatcgcgtgtgaagcctgcttttttatactaagttggcattataaaaaagcattgcttatcaatttgttgcaacgaacaggtcactatcagtcaaaataaaatcattatttgatttcgaattctcatgtttgacagcttatcatcgataagctttaatgcggtagtttatcacagttaaattgctaacgcagtcaggcaccgtgtatgaaatctaacaatgcgctcatcgtcatcctcggcaccgtcaccctggatgctgtaggcataggcttggttatgccggtactgccgggcctcttgcgggatatcgtccattccgacagcatcgccagtcactatggcgtgctgctagcgctatatgcgttgatgcaatttctatgcgcacccgttctcggagcactgtccgaccgctttggccgccgcccagtcctgctcgcttcgctacttggagccactatcgactacgcgatcatggcgaccacacccgtcctgtggatctccggataagtagacagcctgataagtcgcacgaaaaacaggtattgacaacatgaagtaacatgcagtaagatacaaatcgctaggtaacactagcagcgtcaaccgggcgctctagctagagccaagctagcttggccggatccgagattttcaggagctaaggaagctaaaatggagaaaaaaatcactggatataccaccgttgatatatcccaatggcatcgtaaagaacattttgaggcatttcagtcagttgctcaatgtacctataaccagaccgttcagctggatattacggcctttttaaagaccgtaaagaaaaataagcacaagttttatccggcctttattcacattcttgcccgcctgatgaatgctcatccggaattccgtatggcaatgaaagacggtgagctggtgatatgggatagtgttcacccttgttacaccgttttccatgagcaaactgaaacgttttcatcgctctggagtgaataccacgacgatttccggcagtttctacacatatattcgcaagatgtggcgtgttacggtgaaaacctggcctatttccctaaagggtttattgagaatatgtttttcgtctcagccaatccctgggtgagtttcaccagttttgatttaaacgtggccaatatggacaacttcttcgcccccgttttcaccatgggcaaatattatacgcaaggcgacaaggtgctgatgccgctggcgattcaggttcatcatgccgtctgtgatggcttccatgtcggcagaatgcttaatgaattacaacagtactgcgatgagtggcagggcggggcgtaatttttttaaggcagttattggtgcccttaaacgcctggtgctacgcctgaataagtgataataagcggatgaatggcagaaattcgtcgaagcttaacacagaaaaaagcccgcacctgacagtgcgggctttttttttcgaccactgcagtctgttacaggtcactaataccatctaagtagttgattcatagtgactgcatatgttgtgttttacagtattatgtagtctgttttttatgcaaaatctaatttaatatattgatatttatatcattttacgtttctcgttcagcttttttatactaacttgagcgctgcggtgatgtaatgcaggaaagcaggctggagctacccagcctgcagtgaaattaaactgtcgtcgctttcactctttctttatagatgatttttttgatgccatcgttctacgtgaga

SEQ ID NO: 61 - DNA, 64 bp, Artificial Sequence
  Primer P24
aattagctaattttacggatgcagaactcacgctggcgctcaagttagtataaaaaagctgaac

SEQ ID NO: 62 - DNA, 64 bp, Artificial Sequence
  Primer P25
cggaaagcccggtcatttgaccgggcaaggggattatgaagcctgcttttttatactaagttgg

SEQ ID NO: 63 - DNA, 1713 bp, Artificial Sequence
  DNA fragment 22
aattagctaattttacggatgcagaactcacgctggcgctcaagttagtataaaaaagctgaacgagaaacgtaaaatgatataaatatcaatatattaaattagattttgcataaaaaacagactacataatactgtaaaacacaacatatgcagtcactatgaatcaactacttagatggtattagtgacctgtaacagactgcagtggtcgaaaaaaaaagcccgcactgtcaggtgcgggcttttttctgtgttaagcttcgacgaatttctgccattcatccgcttattatcacttattcaggcgtagcaccaggcgtttaagggcaccaataactgccttaaaaaaattacgccccgccctgccactcatcgcagtactgttgtaattcattaagcattctgccgacatggaagccatcacagacggcatgatgaacctgaatcgccagcggcatcagcaccttgtcgccttgcgtataatatttgcccatggtgaaaacgggggcgaagaagttgtccatattggccacgtttaaatcaaaactggtgaaactcacccagggattggctgagacgaaaaacatattctcaataaaccctttagggaaataggccaggttttcaccgtaacacgccacatcttgcgaatatatgtgtagaaactgccggaaatcgtcgtggtattcactccagagcgatgaaaacgtttcagtttgctcatggaaaacggtgtaacaagggtgaacactatcccatatcaccagctcaccgtctttcattgccatacggaattccggatgagcattcatcaggcgggcaagaatgtgaataaaggccggataaaacttgtgcttatttttctttacggtctttaaaaaggccgtaatatccagctgaacggtctggttataggtacattgagcaactgactgaaatgcctcaaaatgttctttacgatgccattgggatatatcaacggtggtatatccagtgatttttttctccattttagcttccttagctcctgaaaatctcggatccggccaagctagcttggctctagctagagcgcccggttgacgctgctagtgttacctagcgatttgtatcttactgcatgttacttcatgttgtcaatacctgtttttcgtgcgacttatcaggctgtctacttatccggagatccacaggacgggtgtggtcgccatgatcgcgtagtcgatagtggctccaagtagcgaagcgagcaggactgggcggcggccaaagcggtcggacagtgctccgagaacgggtgcgcatagaaattgcatcaacgcatatagcgctagcagcacgccatagtgactggcgatgctgtcggaatggacgatatcccgcaagaggcccggcagtaccggcataaccaagcctatgcctacagcatccagggtgacggtgccgaggatgacgatgagcgcattgttagatttcatacacggtgcctgactgcgttagcaatttaactgtgataaactaccgcattaaagcttatcgatgataagctgtcaaacatgagaattcgaaatcaaataatgattttattttgactgatagtgacctgttcgttgcaacaaattgataagcaatgcttttttataatgccaacttagtataaaaaagcaggcttcataatccccttgcccggtcaaatgaccgggctttccg

SEQ ID NO: 64 - DNA, 22 bp, Artificial Sequence
  Primer P26
atgctgaaatatgtcaaccgat

SEQ ID NO: 65 - DNA, 22 bp, Artificial Sequence
  Primer P27
ggtaattgcggttatttctgtt

SEQ ID NO: 66 - DNA, 5172 bp, Artificial Sequence
  DNA fragment 23
atgctgaaatatgtcaaccgatgaaaagcgtcggtagttaagcagaaattaatatcgcttactttaaccaccgcagcacaattagctaattttacggatgcagaactcacgctggcgggacgtttttattgcgtcagggttgacatccgtttttgtatccagtaactctaaaagcatatcgcattcatctggagctgatttaatgactcacatcgttcgctttatcggtctactactactaaacgcatcttctttgcgcggtagacgagtgagcggcatccagcattaagccagcacgcagtcaaacaaaaaacccgcgccattgcgcgggtttttttatgcccgaagcgaggcgctctaaaagagacaaggacccaaaccatgagccagcaagtcattattttcgataccacattgcgcgacggtgaacaggcgttacaggcaagcttgagtgtgaaagaaaaactgcaaattgcgctggcccttgagcgtatgggtgttgacgtgatggaagtcggtttccccgtctcttcgccgggcgattttgaatcggtgcaaaccatcgcccgccaggttaaaaacagccgcgtatgtgcgttagctcgctgcgtggaaaaagatatcgacgtggcggccgaatccctgaaagtcgccgaagccttccgtattcatacctttattgccacttcgccaatgcacatcgccaccaagctgcgcagcacgctggacgaggtgatcgaacgcgctatctatatggtgaaacgcgcccgtaattacaccgatgatgttgaattttcttgcgaagatgccgggcgtacacccattgccgatctggcgcgagtggtcgaagcggcgattaatgccggtgccaccaccatcaacattccggacaccgtgggctacaccatgccgtttgagttcgccggaatcatcagcggcctgtatgaacgcgtgcctaacatcgacaaagccattatctccgtacatacccacgacgatttgggcctggcggtcggaaactcactggcggcggtacatgccggtgcacgccaggtggaaggcgcaatgaacgggatcggcgagcgtgccggaaactgttccctggaagaagtcatcatggcgatcaaagttcgtaaggatattctcaacgtccacaccgccattaatcaccaggagatatggcgcaccagccagttagttagccagatttgtaatatgccgatcccggcaaacaaagccattgttggcagcggcgcattcgcacactcctccggtatacaccaggatggcgtgctgaaaaaccgcgaaaactacgaaatcatgacaccagaatctattggtctgaaccaaatccagctgaatctgacctctcgttcggggcgtgcggcggtgaaacatcgcatggatgagatggggtataaagaaagtgaatataatttagacaatttgtacgatgctttcctgaagctggcggacaaaaaaggtcaggtgtttgattacgatctggaggcgctggccttcatcggtaagcagcaagaagagccggagcatttccgtctggattacttcagcgtgcagtctggctctaacgatatcgccaccgccgccgtcaaactggcctgtggcgaagaagtcaaagcagaagccgccaacggtaacggtccggtcgatgccgtctatcaggcaattaaccgcatcactgaatataacgtcgaactggtgaaatacagcctgaccgccaaaggccacggtaaagatgcgctgggtcaggtggatatcgtcgctaactacaacggtcgccgcttccacggcgtcggcctggctaccgatattgtcgagtcatctgccaaagccatggtgcacgttctgaacaatatctggcgtgccgcagaagtcgaaaaagagttgcaacgcaaagctcaacacaacgaaaacaacaaggaaaccgtgtgatgtcgaagaattaccatattgccgtattgccgggggacggtattggtccggaagtgatgacccaggcgctgaaagtgctggatgccgtgcgcaaccgctttgcgatgcgcatcaccaccagccattacgatgtaggcggcgcagccattgataaccacgggcaaccactgccgcctgcgacggttgaaggttgtgagcaagccgatgccgtgctgtttggctcggtaggcggcccgaagtgggaacatttaccaccagaccagcaaccagaacgcggcgcgctgctgcctctgcgtaagcacttcaaattattcagcaacctgcgcccggcaaaactgtatcaggggctggaagcattctgtccgctgcgtgcagacattgccgcaaacggcttcgacatcctgtgtgtgcgcgaactgaccggcggcatctatttcggtcagccaaaaggccgcgaaggtagcggacaatatgaaaaagcctttgataccgaggtgtatcaccgttttgagatcgaacgtatcgcccgcatcgcgtttgaatctgctcgcaagcgtcgccacaaagtgacgtcgatcgataaagccaacgtgctgcaatcctctattttatggcgggagatcgttaacgagatcgccacggaatacccggatgtcgaactggcgcatatgtacatcgacaacgccaccatgcagctgattaaagatccatcacagtttgacgttctgctgtgctccaacctgtttggcgacattctgtctgacgagtgcgcaatgatcactggctcgatggggatgttgccttccgccagcctgaacgagcaaggttttggactgtatgaaccggcgggcggctcggcaccagatatcgcaggcaaaaacatcgccaacccgattgcacaaatcctttcgctggcactgctgctgcgttacagcctggatgccgatgatgcggcttgcgccattgaacgcgccattaaccgcgcattagaagaaggcattcgcaccggggatttagcccgtggcgctgccgccgttagtaccgatgaaatgggcgatatcattgcccgctatgtagcagaaggggtgtaatcatggctaagacgttatacgaaaaattgttcgacgctcacgttgtgtacgaagccgaaaacgaaaccccactgttatatatcgaccgccacctggtgcatgaagtgacctcaccgcaggcgttcgatggtctgcgcgcccacggtcgcccggtacgtcagccgggcaaaaccttcgctaccatggatcacaacgtctctacccagaccaaagacattaatgcctgcggtgaaatggcgcgtatccagatgcaggaactgatcaaaaactgcaaagaatttggcgtcgaactgtatgacctgaatcacccgtatcaggggatcgtccacgtaatggggccggaacagggcgtcaccttgccggggatgaccattgtctgcggcgactcgcataccgccacccacggcgcgtttggcgcactggcctttggtatcggcacttccgaagttgaacacgtactggcaacgcaaaccctgaaacagggccgcgcaaaaaccatgaaaattgaagtccagggcaaagccgcgccgggcattaccgcaaaagatatcgtgctggcaattatcggtaaaaccggtagcgcaggcggcaccgggcatgtggtggagttttgcggcgaagcaatccgtgatttaagcatggaaggtcgtatgaccctgtgcaatatggcaatcgaaatgggcgcaaaagccggtctggttgcaccggacgaaaccacctttaactatgtcaaaggccgtctgcatgcgccgaaaggcaaagatttcgacgacgccgttgcctactggaaaaccctgcaaaccgacgaaggcgcaactttcgataccgttgtcactctgcaagcagaagaaatttcaccgcaggtcacctggggcaccaatcccggccaggtgatttccgtgaacgacaatattcccgatccggcttcgtttgccgatccggttgaacgcgcgtcggcagaaaaagcgctggcctatatggggctgaaaccgggtattccgctgaccgaagtggctatcgacaaagtgtttatcggttcctgtaccaactcgcgcattgaagatttacgcgcggcagcggagatcgccaaagggcgaaaagtcgcgccaggcgtgcaggcactggtggttcccggctctggcccggtaaaagcccaggcggaagcggaaggtctggataaaatctttattgaagccggttttgaatggcgcttgcctggctgctcaatgtgtctggcgatgaacaacgaccgtctgaatccgggcgaacgttgtgcctccaccagcaaccgtaactttgaaggccgccaggggcgcggcgggcgcacgcatctggtcagcccggcaatggctgccgctgctgctgtgaccggacatttcgccgacattcgcaacattaaataaggagcacaccatggcagagaaatttatcaaacacacaggcctggtggttccgctggatgccgccaatgtcgataccgatgcaatcatcccgaaacagtttttgcagaaagtgacccgtacgggttttggcgcgcatctgtttaacgactggcgttttctggatgaaaaaggccaacagccaaacccggacttcgtgctgaacttcccgcagtatcagggcgcttccattttgctggcacgagaaaacttcggctgtggctcttcgcgtgagcacgcgccctgggcattgaccgactacggttttaaagtggtgattgcgccgagttttgctgacatcttctacggcaatagctttaacaaccagctgctgccggtgaaattaagcgatgcagaagtggacgaactgtttgcgctggtgaaagctaatccggggatccatttcgacgtggatctggaagcgcaagaggtgaaagcgggagagaaaacctatcgctttaccatcgatgccttccgccgccactgcatgatgaacggtctggacagtattgggcttaccttgcagcacgacgacgccattgccgcttatgaagcaaaacaacctgcgtttatgaattaatccccttgcccggtcaaatgaccgggctttccgctatcgtccacgtcatcaaacgtctttaacctttgcggttaaaaataatgcgacaacagaaataaccgcaattacc

SEQ ID NO: 67 - DNA, 1868 bp, Artificial Sequence
  DNA fragment 24
atgctgaaatatgtcaaccgatgaaaagcgtcggtagttaagcagaaattaatatcgcttactttaaccaccgcagcacaattagctaattttacggatgcagaactcacgctggcgctcaagttagtataaaaaagctgaacgagaaacgtaaaatgatataaatatcaatatattaaattagattttgcataaaaaacagactacataatactgtaaaacacaacatatgcagtcactatgaatcaactacttagatggtattagtgacctgtaacagactgcagtggtcgaaaaaaaaagcccgcactgtcaggtgcgggcttttttctgtgttaagcttcgacgaatttctgccattcatccgcttattatcacttattcaggcgtagcaccaggcgtttaagggcaccaataactgccttaaaaaaattacgccccgccctgccactcatcgcagtactgttgtaattcattaagcattctgccgacatggaagccatcacagacggcatgatgaacctgaatcgccagcggcatcagcaccttgtcgccttgcgtataatatttgcccatggtgaaaacgggggcgaagaagttgtccatattggccacgtttaaatcaaaactggtgaaactcacccagggattggctgagacgaaaaacatattctcaataaaccctttagggaaataggccaggttttcaccgtaacacgccacatcttgcgaatatatgtgtagaaactgccggaaatcgtcgtggtattcactccagagcgatgaaaacgtttcagtttgctcatggaaaacggtgtaacaagggtgaacactatcccatatcaccagctcaccgtctttcattgccatacggaattccggatgagcattcatcaggcgggcaagaatgtgaataaaggccggataaaacttgtgcttatttttctttacggtctttaaaaaggccgtaatatccagctgaacggtctggttataggtacattgagcaactgactgaaatgcctcaaaatgttctttacgatgccattgggatatatcaacggtggtatatccagtgatttttttctccattttagcttccttagctcctgaaaatctcggatccggccaagctagcttggctctagctagagcgcccggttgacgctgctagtgttacctagcgatttgtatcttactgcatgttacttcatgttgtcaatacctgtttttcgtgcgacttatcaggctgtctacttatccggagatccacaggacgggtgtggtcgccatgatcgcgtagtcgatagtggctccaagtagcgaagcgagcaggactgggcggcggccaaagcggtcggacagtgctccgagaacgggtgcgcatagaaattgcatcaacgcatatagcgctagcagcacgccatagtgactggcgatgctgtcggaatggacgatatcccgcaagaggcccggcagtaccggcataaccaagcctatgcctacagcatccagggtgacggtgccgaggatgacgatgagcgcattgttagatttcatacacggtgcctgactgcgttagcaatttaactgtgataaactaccgcattaaagcttatcgatgataagctgtcaaacatgagaattcgaaatcaaataatgattttattttgactgatagtgacctgttcgttgcaacaaattgataagcaatgcttttttataatgccaacttagtataaaaaagcaggcttcataatccccttgcccggtcaaatgaccgggctttccgctatcgtccacgtcatcaaacgtctttaacctttgcggttaaaaataatgcgacaacagaaataaccgcaattacc

SEQ ID NO: 68 - DNA, 284 bp, Artificial Sequence
  DNA fragment 25
ggatgtacgtttgtcatgagtctcactctgttgctaattgccgttcgctcctgaacatccactcgatcttcgccttcttccggtttattgtgttttaaccacctgcccgtaaacctggagaaccatcgcgtgtgaagcctgcttttttatactaacttgagcgctgcggtgatgtaatgcaggaaagcaggctggagctacccagcctgcagtgaaattaaactgtcgtcgctttcactctttctttatagatgatttttttgatgccatcgttctacgtgaga

SEQ ID NO: 69 - DNA, 70 bp, Artificial Sequence
  Ptac promoter
ccctgttgacaattaatcatcggctcgtataatgtgtggaattgtgagcggataacaatttcacacagga